European Patent Specification EP 4 043 017 B1, published January 28, 2026. Title: CANCER TREATMENT USING COMBINATIONS OF ERK AND RAF INHIBITORS. Applicant: BIOMED VALLEY DISCOVERIES, INC. The sequence listing filed with the application follows.

SEQUENCE LISTING (47 sequences)

SEQ ID NO: 1 - DNA, 5898 bp, Homo sapiens
cgcctcccttccccctccccgcccgacagcggccgctcgggccccggctctcggttataagatggcggcgctgagcggtggcggtggtggcggcgcggagccgggccaggctctgttcaacggggacatggagcccgaggccggcgccggcgccggcgccgcggcctcttcggctgcggaccctgccattccggaggaggtgtggaatatcaaacaaatgattaagttgacacaggaacatatagaggccctattggacaaatttggtggggagcataatccaccatcaatatatctggaggcctatgaagaatacaccagcaagctagatgcactccaacaaagagaacaacagttattggaatctctggggaacggaactgatttttctgtttctagctctgcatcaatggataccgttacatcttcttcctcttctagcctttcagtgctaccttcatctctttcagtttttcaaaatcccacagatgtggcacggagcaaccccaagtcaccacaaaaacctatcgttagagtcttcctgcccaacaaacagaggacagtggtacctgcaaggtgtggagttacagtccgagacagtctaaagaaagcactgatgatgagaggtctaatcccagagtgctgtgctgtttacagaattcaggatggagagaagaaaccaattggttgggacactgatatttcctggcttactggagaagaattgcatgtggaagtgttggagaatgttccacttacaacacacaactttgtacgaaaaacgtttttcaccttagcattttgtgacttttgtcgaaagctgcttttccagggtttccgctgtcaaacatgtggttataaatttcaccagcgttgtagtacagaagttccactgatgtgtgttaattatgaccaacttgatttgctgtttgtctccaagttctttgaacaccacccaataccacaggaagaggcgtccttagcagagactgccctaacatctggatcatccccttccgcacccgcctcggactctattgggccccaaattctcaccagtccgtctccttcaaaatccattccaattccacagcccttccgaccagcagatgaagatcatcgaaatcaatttgggcaacgagaccgatcctcatcagctcccaatgtgcatataaacacaatagaacctgtcaatattgatgacttgattagagaccaaggatttcgtggtgatggaggatcaaccacaggtttgtctgctaccccccctgcctcattacctggctcactaactaacgtgaaagccttacagaaatctccaggacctcagcgagaaaggaagtcatcttcatcctcagaagacaggaatcgaatgaaaacacttggtagacgggactcgagtgatgattgggagattcctgatgggcagattacagtgggacaaagaattggatctggatcatttggaacagtctacaagggaaagtggcatggtgatgtggcagtgaaaatgttgaatgtgacagcacctacacctcagcagttacaagccttcaaaaatgaagtaggagtactcaggaaaacacgacatgtgaatatcctactcttcatgggctattccacaaagccacaactggctattgttacccagtggtgtgagggctccagcttgtatcaccatctccatatcattgagaccaaatttgagatgatcaaacttatagatattgcacgacagactgcacagggcatggattacttacacgccaagtcaatcatccacagagacctcaagagtaataatatatttcttcatgaagacctcacagtaaaaataggtgattttggtctagctacagtgaaatctcgatggagtgggtcccatcagtttgaacagttgtctggatccattttgtggatggcaccagaagtcatcagaatgcaagataaaaatccatacagctttcagtcagatgtatatgcatttggaattgttctgtatgaattgatgactggacagttaccttattcaaacatcaacaacagggaccagataatttttatggtgggacgaggatacctgtctccagatctcagtaaggtacggagtaactgtccaaaagccatgaagagattaatggcagagtgcctcaaaaagaaaagagatgagagaccactctttccccaaattctcgcctctattgagctgctggcccgctcattgccaaaaattcaccgcagtgcatcagaaccctccttgaatcgggctggtttccaaacagaggattttagtctatatgcttgtgcttctccaaaaacacccatccaggcagggggatatggtgcgtttcctgtccactgaaacaaatgagtgagagagttcaggagagtagcaacaaaaggaaaataaatgaacatatgtttgcttatatgttaaattgaataaaatactctctttttttttaaggtgaaccaaagaacacttgtgtggttaaagactagatataatttttccccaaactaaaatttatacttaacattggatttttaacatccaagggttaaaatacatagacattgctaaaaattggcagagcctcttctagaggctttactttctgttccgggtttgtatcattcacttggttattttaagtagtaaacttcagtttctcatgcaacttttgttgccagctatcacatgtccactagggactccagaagaagaccctacctatgcctgtgtttgcaggtgagaagttggcagtcggttagcctgggttagataaggcaaactgaacagatctaatttaggaagtcagtagaatttaataattctattattattcttaataatttttctataactatttctttttataacaatttggaaaatgtggatgtcttttatttccttgaagcaataaactaagtttctttttataaaaacgcctcccttccccctccccgcccgacagcggccgctcgggccccggctctcggttataagatggcggcgctgagcggtggcggtggtggcggcgcggagccgggccaggctctgttcaacggggacatggagcccgaggccggcgccggcgccggcgccgcggcctcttcggctgcggaccctgccattccggaggaggtgtggaatatcaaacaaatgattaagttgacacaggaacatatagaggccctattggacaaatttggtggggagcataatccaccatcaatatatctggaggcctatgaagaatacaccagcaagctagatgcactccaacaaagagaacaacagttattggaatctctggggaacggaactgatttttctgtttctagctctgcatcaatggataccgttacatcttcttcctcttctagcctttcagtgctaccttcatctctttcagtttttcaaaatcccacagatgtggcacggagcaaccccaagtcaccacaaaaacctatcgttagagtcttcctgcccaacaaacagaggacagtggtacctgcaaggtgtggagttacagtccgagacagtctaaagaaagcactgatgatgagaggtctaatcccagagtgctgtgctgtttacagaattcaggatggagagaagaaaccaattggttgggacactgatatttcctggcttactggagaagaattgcatgtggaagtgttggagaatgttccacttacaacacacaactttgtacgaaaaacgtttttcaccttagcattttgtgacttttgtcgaaagctgcttttccagggtttccgctgtcaaacatgtggttataaatttcaccagcgttgtagtacagaagttccactgatgtgtgttaattatgaccaacttgatttgctgtttgtctccaagttctttgaacaccacccaataccacaggaagaggcgtccttagcagagactgccctaacatctggatcatccccttccgcacccgcctcggactctattgggccccaaattctcaccagtccgtctccttcaaaatccattccaattccacagcccttccgaccagcagatgaagatcatcgaaatcaatttgggcaacgagaccgatcctcatcagctcccaatgtgcatataaacacaatagaacctgtcaatattgatgacttgattagagaccaaggatttcgtggtgatggaggatcaaccacaggtttgtctgctaccccccctgcctcattacctggctcactaactaacgtgaaagccttacagaaatctccaggacctcagcgagaaaggaagtcatcttcatcctcagaagacaggaatcgaatgaaaacacttggtagacgggactcgagtgatgattgggagattcctgatgggcagattacagtgggacaaagaattggatctggatcatttggaacagtctacaagggaaagtggcatggtgatgtggcagtgaaaatgttgaatgtgacagcacctacacctcagcagttacaagccttcaaaaatgaagtaggagtactcaggaaaacacgacatgtgaatatcctactcttcatgggctattccacaaagccacaactggctattgttacccagtggtgtgagggctccagcttgtatcaccatctccatatcattgagaccaaatttgagatgatcaaacttatagatattgcacgacagactgcacagggcatggattacttacacgccaagtcaatcatccacagagacctcaagagtaataatatatttcttcatgaagacctcacagtaaaaataggtgattttggtctagctacagtgaaatctcgatggagtgggtcccatcagtttgaacagttgtctggatccattttgtggatggcaccagaagtcatcagaatgcaagataaaaatccatacagctttcagtcagatgtatatgcatttggaattgttctgtatgaattgatgactggacagttaccttattcaaacatcaacaacagggaccagataatttttatggtgggacgaggatacctgtctccagatctcagtaaggtacggagtaactgtccaaaagccatgaagagattaatggcagagtgcctcaaaaagaaaagagatgagagaccactctttccccaaattctcgcctctattgagctgctggcccgctcattgccaaaaattcaccgcagtgcatcagaaccctccttgaatcgggctggtttccaaacagaggattttagtctatatgcttgtgcttctccaaaaacacccatccaggcagggggatatggtgcgtttcctgtccactgaaacaaatgagtgagagagttcaggagagtagcaacaaaaggaaaataaatgaacatatgtttgcttatatgttaaattgaataaaatactctctttttttttaaggtgaaccaaagaacacttgtgtggttaaagactagatataatttttccccaaactaaaatttatacttaacattggatttttaacatccaagggttaaaatacatagacattgctaaaaattggcagagcctcttctagaggctttactttctgttccgggtttgtatcattcacttggttattttaagtagtaaacttcagtttctcatgcaacttttgttgccagctatcacatgtccactagggactccagaagaagaccctacctatgcctgtgtttgcaggtgagaagttggcagtcggttagcctgggttagataaggcaaactgaacagatctaatttaggaagtcagtagaatttaataattctattattattcttaataatttttctataactatttctttttataacaatttggaaaatgtggatgtcttttatttccttgaagcaataaactaagtttctttttataaaaa

SEQ ID NO: 2 - protein, 765 aa, Homo sapiens
AALSGGGGGGAEPGQALFNGDMEPEAGAGAGAAASSAADPAIPEEVWNIKQMIKLTQEHIEALLDKFGGEHNPPSIYLEAYEEYTSKLDALQQREQQLLESLGNGTDFSVSSSASMDTVTSSSSSSLSVLPSSLSVFQNPTDVARSNPKSPQKPIVRVFLPNKQRTVVPARCGVTVRDSLKKALMMRGLIPECCAVYRIQDGEKKPIGWDTDISWLTGEELHVEVLENVPLTTHNFVRKTFFTLAFCDFCRKLLFQGFRCQTCGYKFHQRCSTEVPLMCVNYDQLDLLFVSKFFEHHPIPQEEASLAETALTSGSSPSAPASDSIGPQILTSPSPSKSIPIPQPFRPADEDHRNQFGQRDRSSSAPNVHINTIEPVNIDDLIRDQGFRGDGGSTTGLSATPPASLPGSLTNVKALQKSPGPQRERKSSSSSEDRNRMKTLGRRDSSDDWEIPDGQITVGQRIGSGSFGTVYKGKWHGDVAVKMLNVTAPTPQQLQAFKNEVGVLRKTRHVNILLFMGYSTKPQLAIVTQWCEGSSLYHHLHIIETKFEMIKLIDIARQTAQGMDYLHAKSIIHRDLKSNNIFLHEDLTVKIGDFGLATVKSRWSGSHQFEQLSGSILWMAPEVIRMQDKNPYSFQSDVYAFGIVLYELMTGQLPYSNINNRDQIIFMVGRGYLSPDLSKVRSNCPKAMKRLMAECLKKKRDERPLFPQILASIELLARSLPKIHRSASEPSLNRAGFQTEDFSLYACASPKTPIQAGGYGAFPVH

SEQ ID NO: 3 - DNA, 3906 bp, Rattus norvegicus
atggcggcgctgagtggcggcggtggcagcagcagcggtggcggtggcggcggcggcggcggcggtggtggcggcggcggcggcggcgccgaacagggacaggctctgttcaatggcgacatggagccggaggccggcgctggcgccgcggcctcttcggccgcggacccggccattcctgaagaggtgtggaatatcaagcaaatgattaagttgacacaggaacatatagaggccctattggacaagtttggtggggagcataacccaccgtcaatatacctggaggcctatgaagagtacaccagcaagctagatgcccttcagcagagagagcagcagctgttggaatccctggtttttcaaactcccacagatgtatcacggaacaaccccaagtcaccacagaaacctatcgttcgtgtcttcctgcccaacaaacagaggacagtggtgcccgcaagatgtggtgtaacggtccgagacagtctaaagaaagcactaatgatgaggggtctcatcccagagtgctgtgctgtttacagaattcaggacggagagaagaaaccaattggctgggacactgacatttcctggcttactggagaggagctacatgttgaagtactagagaatgttcctctgacaacccacaacttcgtacggaaaacttttttcaccttagcattttgtgacttttgccgaaagctgcttttccagggtttccgctgtcaaacatgtggttataagtttcaccagcgttgtagtacagaggttccactgatgtgtgttaattatgaccaacttgatttgctgtttgtctccaagttctttgagcatcacccagtaccacaggaggaggccttctcagcagagactacccttccatctggatgctcttccgcacccccctcagactctattgggccccaaatcctcaccagtccatctccttcaaaatccattccaattccacagcccttccggccagcagatgaagatcatcgcaatcagtttgggcaacgagaccgctcctcctccgctcccaatgttcatataaacacaatcgaacctgtcaatattgatgaaaaattcccagaagtggaattacaggatcaaagggatttgattagagaccaggggtttcgtggggatggagcccctttgaaccagctgatgcgctgtcttcggaaataccaatcccggactcccagccccctcctccattctgtccccagtgaaatagtgtttgattttgagcctggcccagtgttcagagggtcaaccacaggcttgtcggccaccccacctgcctcattacctggctcactcactaacgtgaaagccttacagaaatctccaggacctcagcgggaaaggaagtcctcctcctcctcctcctccacggaagacagaagtcggatgaaaacacttggtagaagagattcaagtgatgattgggagattcctgatggacagattacagtgggacagagaattggatctgggtcctttggaactgtctacaagggaaagtggcatggcgacgtggcagtgaaaatgctgaatgtgacagcacccacacctcagcagttacaggccttcaaaaacgaagtcggagtactcaggaaaactcgacatgtgaacatcctccttttcatgggctattctacaaagccacagctggctattgttacacagtggtgtgaaggctccagcttatatcaccatctccacatcattgagaccaaatttgagatgatcaaacttatagatattgcacggcagactgcacagggcatggattacttacacgccaagtcaatcatccacagagacctcaagagtaataatatatttcttcatgaagacctcacggtaaaaataggtgactttggtttagccacagtgaagtcccgatggagtgggtcccatcagtttgaacagttgtctggatctattttgtggatggcacccgaagtaatcagaatgcaagataaaaacccatatagctttcagtcagacgtgtatgcatttgggattgttctgtatgaactgatgactggtcagctaccttattcaaacatcaacaacagggatcagataatttttatggtgggacgaggatacctatctccagatctcagtaaggtacggagtaactgtccaaaagccatgaagagattaatggcagagtgcctcaaaaagaaaagagacgagagaccactctttccccaaattctcgcctctattgagctgctggcccgctcattgccaaaaattcaccgcagtgcatcagaaccctccttgaatcgggctggtttccaaacagaagattttagtctgtatgcttgtgcttctccaaaaacacccatccaagcagggggatatggagaatttgcagccttcaagtagccactccatcatggcagcatctactctttatttcttaagtcttgtgttcatacaatttgttaacatcaaaacacagttctgttcctcaaattttttttaaagatacaaaattttcaatgcataagctcgtgtggaacagaatggaatttcctattcaacaaaagagggaagaatgttttaggaaccagaattctctgctgcccgtgtttcttcttcaacacaaatatcatgtgcatacaactctgcccattcccaagaagaaagaggagagaccccgaattctgcccttttggtggtcaggcatgatggaaagaatttgctgctgcagcttgggaaaaattgctatggaaagtctgccagtcaactttgcccttctaaccaccagatccatttgtggctggtcatctgatggggcgatttcaatcaccaagcatcgttcttgcctgttgtgggattatgtcgtggagcactttccctatccaccaccgttaatttccgagggatggagtaaatgcagcataccctttgtgtagcacctgtccagtcctcaaccaatgctatcacagtgaagctctttaaatttaagtggtgggtgagtgttgaggagagactgccttgggggcagagaaaaggggatgctgcatcttcttcctcacctccagctctctcacctcgggttgccttgcacactgggctccgcctaaccactcgggctgggcagtgctggcacacattgccgccttttctcattgggtccagcaattgagcagagggttgggggattgtttcctccacaatgtagcaaattctcaggaaaatacagtccatatcttcctctcagctcttccagtcaccaaatacttacgtggctcctttgtccaggacataaaacaccgtggacaacacctaattaaaagcctacaaaactgcttactgacagttttgaatgtgagacatttgtgtaatttaaatgtaaggtacaggtcttaatttcttctattaagtttcttctatttttatttaaacgaagaaaataattttcaggtttaattggaataaacgaatacttcccaaaagactatataccctgaaaattatatttttgttaattgtaaacaacttttaaaaaatggttattatccttttctctacctaaaattatgggaaatcttagcataatgacaattatttatactttttaaataaatggtacttgctggatccacactaacatctttgctaacattcccattgtttcttccaacttcactcctacactacatcctccatcctctttctagtcttttatctataatatgcaacctaaaataaaagtggtggtgtctccattcattcttcttcttccttttttccccaagcctggtcttcaaaaggttgggtaatttagtagctgagttccctaggtagaaatagaactattagggacattggggttgtaggaaagcgtgaggcctgtcaccagttgttctt

SEQ ID NO: 4 - protein, 804 aa, Rattus norvegicus
MAALSGGGGSSSGGGGGGGGGGGGGGGGGAEQGQALFNGDMEPEAGAGAAASSAADPAIPEEVWNIKQMIKLTQEHIEALLDKFGGEHNPPSIYLEAYEEYTSKLDALQQREQQLLESLVFQTPTDVSRNNPKSPQKPIVRVFLPNKQRTVVPARCGVTVRDSLKKALMMRGLIPECCAVYRIQDGEKKPIGWDTDISWLTGEELHVEVLENVPLTTHNFVRKTFFTLAFCDFCRKLLFQGFRCQTCGYKFHQRCSTEVPLMCVNYDQLDLLFVSKFFEHHPVPQEEAFSAETTLPSGCSSAPPSDSIGPQILTSPSPSKSIPIPQPFRPADEDHRNQFGQRDRSSSAPNVHINTIEPVNIDEKFPEVELQDQRDLIRDQGFRGDGAPLNQLMRCLRKYQSRTPSPLLHSVPSEIVFDFEPGPVFRGSTTGLSATPPASLPGSLTNVKALQKSPGPQRERKSSSSSSSTEDRSRMKTLGRRDSSDDWEIPDGQITVGQRIGSGSFGTVYKGKWHGDVAVKMLNVTAPTPQQLQAFKNEVGVLRKTRHVNILLFMGYSTKPQLAIVTQWCEGSSLYHHLHIIETKFEMIKLIDIARQTAQGMDYLHAKSIIHRDLKSNNIFLHEDLTVKIGDFGLATVKSRWSGSHQFEQLSGSILWMAPEVIRMQDKNPYSFQSDVYAFGIVLYELMTGQLPYSNINNRDQIIFMVGRGYLSPDLSKVRSNCPKAMKRLMAECLKKKRDERPLFPQILASIELLARSLPKIHRSASEPSLNRAGFQTEDFSLYACASPKTPIQAGGYGEFAAFK

SEQ ID NO: 5 - DNA, 9728 bp, Mus musculus
ccctcaggctcggctgcgccggggccgccggcgggttccagaggtggcctccgccccggccgctccgcccacgccccccgcgcctccgcgcccgcctccgcccgccctgcgcctcccttccccctccccgccccgcggcggccgctcggcccggctcgcgcttcgaagatggcggcgctgagtggcggcggtggcagcagcagcggtggcggcggcggcggtggcggcggcggtggcggtggcgacggcggcggcggcgccgagcagggccaggctctgttcaatggcgacatggagccggaggccggcgctggcgccgcggcctcttcggctgcggacccggccattcctgaagaggtatggaatatcaagcaaatgattaagttgacacaggaacatatagaggccctattggacaaatttggtggagagcataacccaccatcaatatacctggaggcctatgaagagtacaccagcaagctagatgcccttcagcaaagagaacagcagcttttggaatccctggtttttcaaactcccacagatgcatcacggaacaaccccaagtcaccacagaaacctatcgttagagtcttcctgcccaacaaacagaggacagtggtacccgcaagatgtggtgttacagttcgagacagtctaaagaaagcactgatgatgagaggtctcatcccagaatgctgtgctgtttacagaattcaggatggagagaagaaaccaattggctgggacacggacatttcctggcttactggagaggagttacatgttgaagtactggagaatgtcccacttacaacacacaactttgtacggaaaacttttttcaccttagcattttgtgacttttgccgaaagctgcttttccagggtttccgttgtcaaacatgtggttataaatttcaccagcgttgtagtacagaggttccactgatgtgtgtaaattatgaccaacttgatttgctgtttgtctccaagttctttgagcatcacccagtaccacaggaggaggcctccttcccagagactgcccttccatctggatcctcttccgcacccccctcagactctactgggccccaaatcctcaccagtccatctccttcaaaatccattccaattccacagcccttccgaccagcagatgaagatcatcgcaatcagtttgggcaacgagaccggtcctcctcagctcccaatgttcatataaacacaattgagcctgtgaatatcgatgaaaaattcccagaagtggaattacaggatcaaagggatttgattagagaccaggggtttcgtggtgatggagcccccttgaaccaactgatgcgctgtcttcggaaataccaatcccggactcccagccccctcctccattctgtccccagtgaaatagtgtttgattttgagcctggcccagtgttcagagggtcaaccacaggcttgtccgccaccccgcctgcctcattacctggctcactcactaacgtgaaagccttacagaaatctccaggtcctcagcgggaaaggaagtcatcttcttcctcatcctcggaggacagaagtcggatgaaaacacttggtagaagagattcaagtgatgactgggagattcctgatggacagattacagtgggacagagaattggatctgggtcatttggaactgtctacaagggaaagtggcatggtgatgtggcagtgaaaatgttgaatgtgacagcacccacacctcaacagctacaggccttcaaaaatgaagtaggagtgctcaggaaaactcgacatgtgaatatcctccttttcatgggctattctacaaagccacaactggcaattgttacacagtggtgtgagggctccagcttatatcaccatctccacatcattgagaccaaatttgagatgatcaaacttatagatattgctcggcagactgcacagggcatggattacttacacgccaagtcaatcatccacagagacctcaagagtaataatatatttcttcatgaagacctcacggtaaaaataggtgactttggtctagccacagtgaaatctcggtggagtgggtcccatcagtttgaacagttgtctggatctattttgtggatggcaccagaagtaatcagaatgcaagataaaaacccgtatagctttcagtcagacgtgtatgcgtttgggattgttctgtacgaactgatgaccggccagctaccttattcaaacatcaacaacagggatcagataatttttatggtgggacgaggatacctatctccagatctcagtaaggtacggagtaactgtccaaaagccatgaagagattaatggcagagtgcctcaaaaagaaaagagacgagagaccactctttccccaaattctcgcctccattgagctgctggcccgctcattgccaaaaattcaccgcagtgcatcagaaccttccttgaatcgggctggtttccaaacagaagattttagtctgtatgcttgtgcttctccgaaaacacccatccaagcagggggatatggagaatttgcagccttcaagtagccagtccatcatggcagcatctactctttatttcttaagtcttgtgttcatacagtttgttaacatcaaaacacagttctgttcctcaaaaaattttttaaagatacaaaattttcaatgcataagttcatgtggaacagaatggaatttcctattcaacaaaagagggaagaatgttttaggaaccagaattctctgctgcccgtgtttcttcttcaacataactatcacgtgcatacaagtctgcccattcccaagaagaaagaggagagaccctgaattctgcccttttggtggtcaggcatgatggaaagaatttgctgctgcagcttgggaaaattgctatggaaagtctgccagtcgactttgcccttctaaccaccagatcagcctgtggctggtcatctgatggggcgatttccatcaccaagcatcgttcttgcctattctgggattatgttgtggagcactttccctgtccagcaccgttcatttctgagggatggagtaaatgcagcattcccttgtgtagcgcctgttcagtcctcagcagctgctgtcacagcgaagctttttacagttaagtggtgggggagagttgaggagagcctgcctcggggcagagaaaagggggtgctgcatcttcttcctcacctccagctctctcacctcgggttgccttgctcactgggctccgcctaaccactcaggctgctcagtgctggcacacattgccttcttttctcattgggtccagcaattgaggagagggttgggggattgtttcctcctcaatgtagcaaattctcaggaaaatacagtccatatcttcctctcagctcttccagtcaccaaatacttacgtggctcctttgtccaggacataaaacaccgtggacaacacctaattaaaagcctacaaaactgcttactgacagttttgaatgtgagacacttgtgtaatttaaatgtaaggtacaggttttaatttctgagtttcttctatttttatttaaaagaagaaaataattttcagttttaattggaataaatgagtacttcccacaagactatataccctgaaaattatatttttgttaattgtaaacaacttttaaagaataattattatccttttctctacctaaaaattatggggaatcttagcataatgacaattatttatactttttaaataaatggtacttgctggatccacactaacatctttgctaacaatcccattgtttcttccaacttaactcctacactacatcctacatcctctttctagtcttttatctataatatgcaacctaaaataaacgtggtggcgtctccattcattctccctcttcctgttttccccaagcctggtcttcaaaaggttgggtaatcggtccctgagctccctagctggcaatgcaactattagggacattggagttgcaggagagcaggaagcctgtccccagctgttcttctagaaccctaaatcttatctttgcacagatcaaaagtatcacctcgtcacagttctccttagcctttacttacaggtaatataaataaaaatcaccatagtagtaaagaaaacaactggatggattgatgaccagtacctctcagagccaggaatcttgaatctccaggatttatacgtgcaaatttaaggagatgtacttagcaacttcaagccaagaacttccaaaatactagcgaatctaaaataaaatggaattttgagttatttttaaagttcaaattataattgataccactatgtatttaagcctactcacagcaagttagatggattttgctaaactcattgccagactgtggtggtggtggtggtagtgtgcacctttaatccaagcaactcagcaatcagaatgaggtaaatctctgtgaatacaaggcctgcctagtctgcagcgctagttccaggatagccagggctacacacacaaaaaccctctctcaaaaaaaacaaaattaattagttgataataaaaaataactaaagtatcatcaaaggaaggcctactggaagttttatatattcccagtaaattgaaaaatattctgaagttattaaccagttagcaacaatgtgtttttaagtcttacataaacagagcaaagtcttcaaatgtttcagagctgagaagataattgtgcttgatatgaaaaatagcctctccatatgatgtgccacattgaaaggcgtcattacccttttaaatacttcttaatgtggctttgttccctttacccaggattagctagaaagagctaggtaggcttcggccacagttgcacatttcgggcctgctgaagaatgggagctttgaaggctggccttggtggaggagcccctcagtgctggagggtggggcgtgtacgcagcatggaagtggtctagacagagtgcaaagggacagacttctttctcattttagtatagggtgatgtctcacttgaaatgagaaagtagagttgatattaaacgaagctgtgcccagaaaccaggctcagggtattgtgagattttctttttaaatagagaatataaaagatagaaataaatatttaaaccttccttcttattttctatcaaatagattttttttatcatttgcaaacaacataaaaaaaggtttcttttgtggggttttctttccttcttttttttttttttttttttttaagactgcagataatcttgttgagctcctcggaaaatacaaggaagtccgtgtttgtgcagagcgctttatgagtaactgtatagacagtgtggctgcttcactcatcccagagggctgcagctgtcggcccatgaagtggctgcagtgcctcgtgagatctgctttgttttgtttggagtgaagtctttgaaaggtttgagtgcaactatataggactgtttttaaataagtagtattcctcatgaactttctcattgttaagctacaggacccaaactctaccactaagatattattaacctcaaaatgtagtttatagaaggaatttgcaaatagaatatccagttcgtacttatatgcatcttcaacaaagattctctgtgacttgttggatttggttcctgaacagcccatttctgtatttgaggttaggagggcataatgaggcatcctaaaagacaatctgatataaactgtatgctagatgtatgctggtaggggagaaagcattctgtaaagacatgatttaagacttcagctctgtcaaccagaaaccttgtaaatacttcctgtcttggtgcagccccgcccctttgatcacacgatgttgtcttgtgcttgtcagacactgtcagagctgctgttcgtccctctgcagatctcacctgtccccactgcacacccacctcctgcctcttgcagacctcagcatctagctttagttggaaacagttcagggttcaggtgacttcttaaaaaaaaaaaaaaaccctacctcctcagaatgaggtaatgaatagttatttatttaaagtatgaagagtcaggagcgctcgaacatgaaggtgatttaagatggttcctttcgtgtgtattgtagctgagcacttgtttttgtcctaaagggcattatacatttaagcagtgattctgtttaaagatgtttttctttaaaggtgtagctcagagtatctgttgttggaattggtgccagagtctgcttaatagatttcagaatcctaagcttaagtcagtcgcatgaagttaagtagttatggtaacactttgctagccatgatataattctactttttaggagtaggtttggcaaaactgtatgccttcaaagtgagttggccacagctttgtcacatgcacagatactcatctgaagagactgcccagctaagagggcggaaggatacccttttttcctacgattcgcttctttgtccacgttggcattgttagtactagtttatcagcaccttgaccagcagatgtcaaccaataagctatttttaaaaccatagccagagatggagaggtcactgtgagtagaaacagcaggacgcttacaggagtgaaatggtgtagggaggctctagaaaaatatcttgacaatttgccaaatgatcttactgtgccttcatgatgcaataaaaaagctaacattttagcagaaatcagtgatttacgaagagagtggccagtctggtttaactcagctgggataatatttttagagtgcaatttagactgcgaagataaatgcactaaagagtttatagccaattcacatttgaaaaataagaaaatggtaaattttcagtgaaatatttttttaaagcacataatccctagtgtagccagaaatatttaccacatagagcagctaggctgagatacagtccagtgacatttctagagaaaccttttctactcccacgggctcctcaaagcatggaaattttatacaaaatgtttgacattttaagatactgctgtagtttagttttgaaatagtatgtgctgagcagcaatcatgtactaactcagagagagaaaacaacaacaaattgtgcatctgatttgttttcagagaaatgctgccaacttagatactgagttctcagagcttcaagtgtaaacttgcctcccaagtcctgtttgcaaatgaagttggctagtgctactgactgctccagcacatgatggaaggcagggggctgtctctgaagtgtcttctataaagggacaatagaatagtgagagacctggtcagtgtgtgtcagctggacactccatgctatgggacttgcatcttctgtcctcaccatccccaagacattgtgctttcctcagttgtcctctagctgtttcactcagacaccaagatgaattactgatgccagaaggggccaaaatggccagtgtgttttgggggttgtatcagttgactggacaataactttaatagtttcagatcatttatttttacttccattttgacagacatttaaatggaaatttagtcctaacttttgtcatttgaaaggaaaaattaacagttcctataagatacttttgaggtggaatctgacatcctaattttttttcttttcagtgggtttgcagcgagggtcttgtatgcactaggcaagggttctaccactaagccacatttcccaggaaataaaatgttaacagttaaaacatacacacaaatacacaaacaccttattaccactttagtaaagtgagagatgtgcgtcctttgtctcagtctccacgatttcagctgccccttgtatgaataactcagtctcgctaaactgtttacttttatttacctggtttgactagttgcagctatataaccagttgtgcatgaggacaacagccagtgtgtttgttttgtttttggttttttgtggtacattttttgtaaagaattctgtagattgaagtgctctttgaaaacagaactgagatatatttattcttgttagcatcaaaaaacattttgtgcaaatgatttgcttttcctggcaggctgagtaccatatccagcgcccacaattgcgggttcccatctaccatgtccacaggggagacagacgggaagcacatgaggggtgtgtttacagagttgtaggagttatgtagttctcttgttgccttggaaatcactgttgttttaagactgttgaacccgtgtgtttggctgggctgtgagttacatgaagaaactgcaaactagcatatgcagacaaagctcacagactaggcgtaaatggaggaaaatggaccaaaataaggcagggtgacacataaaccttgggcttcggagaaaactaagggtggagatgaactataatcacctgaatacaatgtaagagtgcaataagtgtgcttattctaagctgtgaacttcttttaaatcattcctttctaatacatttatgtatgttccattgctgactaaaaccagctatgagaacatatgcctttttattcatgttaactaccagtttaagtggctaaccttaatgtcttatttatcttcattttgtattagtttacataccaggtatgtgtgtgtgctgtactcttcttccctttatttgaaaacacttttcactgggtcatctccttggccattccacaacacaactttggtttggctttcaatgtcaccttatttgatggcctgtgtcccagtagcagaatttatggtattcccattgctggctgctcttccgaccctttgcttctacagcacttgtctctcctaagatagtcagaaactaactgatcaggggatggacttcaccattcatcgtgtctcttcaattctattaaatagaccactcttgggctttagaccaggaaaaaggagacagctctagccatctaccaagcctcaccctaaaaggtcacccgtacttcttggtctgaggacaagtctccactccagtaagggagaggggaggaaatgcttcctgtttgaaatgcagtgaattcctatggctcctgtttcaccacccgcacctatggcaacccatatacattcctcttgtctgtaactgccaaaggttgggtttatgtcacttcagttccactcaagcattgaaaaggttctcatggagtctggggtgtgcccagtgaaaagatggggactttttcattatccacagacctctctatacctgctttgcaaaaattataatggagtaactatttttaaagcttatttttcaattcataagaaaaagacatttattttcaatcaaatggatgatgtctcttatcccttatccctcaatgtttgcttgaattttgtttgttccctatacctactccctaattctttagttccttcctgctcaggtcccttcatttgtactttggagtttttctcatgtaaatttgtataatggaaaatattgttcagtttggatagaaagcatggagaaataaataaaaaaagatagctgaaaatcaaattgaagaaatttatttctgtgtaaagttatttaaaaactctgtattatatttaaagaaaaaagcccaaccccccaaaaagtgctatgtaattgatgtgaatatgcgaatactgctataataaagattgactgcatggagaaa

SEQ ID NO: 6 - protein, 804 aa, Mus musculus
MAALSGGGGSSSGGGGGGGGGGGGGDGGGGAEQGQALFNGDMEPEAGAGAAASSAADPAIPEEVWNIKQMIKLTQEHIEALLDKFGGEHNPPSIYLEAYEEYTSKLDALQQREQQLLESLVFQTPTDASRNNPKSPQKPIVRVFLPNKQRTVVPARCGVTVRDSLKKALMMRGLIPECCAVYRIQDGEKKPIGWDTDISWLTGEELHVEVLENVPLTTHNFVRKTFFTLAFCDFCRKLLFQGFRCQTCGYKFHQRCSTEVPLMCVNYDQLDLLFVSKFFEHHPVPQEEASFPETALPSGSSSAPPSDSTGPQILTSPSPSKSIPIPQPFRPADEDHRNQFGQRDRSSSAPNVHINTIEPVNIDEKFPEVELQDQRDLIRDQGFRGDGAPLNQLMRCLRKYQSRTPSPLLHSVPSEIVFDFEPGPVFRGSTTGLSATPPASLPGSLTNVKALQKSPGPQRERKSSSSSSSEDRSRMKTLGRRDSSDDWEIPDGQITVGQRIGSGSFGTVYKGKWHGDVAVKMLNVTAPTPQQLQAFKNEVGVLRKTRHVNILLFMGYSTKPQLAIVTQWCEGSSLYHHLHIIETKFEMIKLIDIARQTAQGMDYLHAKSIIHRDLKSNNIFLHEDLTVKIGDFGLATVKSRWSGSHQFEQLSGSILWMAPEVIRMQDKNPYSFQSDVYAFGIVLYELMTGQLPYSNINNRDQIIFMVGRGYLSPDLSKVRSNCPKAMKRLMAECLKKKRDERPLFPQILASIELLARSLPKIHRSASEPSLNRAGFQTEDFSLYACASPKTPIQAGGYGEFAAFK

SEQ ID NO: 7 - DNA, 2232 bp, Oryctolagus cuniculus
atggggaatgtgtggaatatcaaacaaatgattaagttgacacaggagcatatagaggccctattggacaaatttggtggggagcataatccaccatcaatatatctggaggcctacgaagaatacaccagcaagctagatgccctccaacaaagagaacagcagttattggaatccctagtttttcaaaatcccacagatgtgtcacggagcaaccccaagtcaccacaaaaacctattgttagagtcttcctgcccaacaaacagaggacagtggtacctgcaagatgtggagttacggttcgagacagtctaaagaaagcgctgatgatgagaggtctgatcccagaatgctgtgctgtttacagaattcaggatggagagaagaagccaattggctgggacactgatatttcctggctcactggagaagagctgcatgtggaagtgttagagaatgtcccactcaccacacataactttgtacggaaaacttttttcaccttagcattttgtgacttctgtagaaagctgcttttccagggtttccgctgtcaaacatgtggctacaaatttcaccagcgttgtagtacggaagttccactgatgtgtgttaattatgaccaacttgatttgctgtttgtctccaagttctttgaacaccacccagtaccacaggaggaggcctccttagcagagactgccctcacatctgggtcatcgccttccgcacctccctcagactctattgggcaccaaattctcaccagtccgtccccttcaaaatccattccgattccacagtccttccgaccagcagatgaagatcatcgaaatcagtttgggcaacgagaccggtcttcatcagcgcctaatgttcacattaacacaatagaacctgtcaatattgatgaaaaattcccagaagtggaattacaggatcaaagggacttgattagagaccaagggtttcgtggtgatggagcccctttgaaccagctgatgcgctgtcttcggaaataccaatcccggactcccagtcccctcctaccttctgtccccagtgacatagtgtttgattttgagcctggcccagtgttcagaggatcgaccacgggtttgtctgccactccccctgcctcattacctggctcactcactagtgtgaaagctgtacagagatccccaggacctcagcgagagaggaagtcgtcttcctcctcagaagacaggaatcgaatgaaaactcttggtagacgggattcaagtgatgattgggagattcctgatgggcagatcaccgtgggacagagaattggatctggatcatttggaaccgtctacaagggaaaatggcacggtgatgtggcagtaaaaatgttgaatgtgacagcacctacacctcagcagttacaggccttcaaaaatgaagtaggagtactcaggaaaacacgacatgtgaatatcctacttttcatgggctattccacaaagccacagctggctattgttacccagtggtgtgagggctccagtttatatcaccatctccacatcattgagaccaaattcgagatgatcaaacttatagatattgcacggcagactgcacagggcatggattacttacacgccaagtcaatcatccacagagacctcaagagtaataatatatttcttcatgaagacctcacagtaaaaataggtgattttggtctagccacagtgaaatctcgatggagtgggtcccatcagtttgaacaattgtctggatccattttgtggatggcaccagaagtaatcagaatgcaagacaaaaacccatatagctttcagtcagatgtatatgcatttgggattgttctgtatgaattgatgactgggcagttaccttactcaaacatcaacaacagggaccagatcatttttatggtgggacgtggctacctgtctccagacctcagtaaggtacggagtaactgtccgaaagccatgaagagattaatggcagagtgcctcaaaaagaaaagagatgagagaccactctttccccaaattctcgcctccattgagctgctggcccgctcattgccaaaaatccaccgcagtgcatcagaaccctccttgaatcgggctggtttccagacagaggattttagtctatatgcttgtgcttctccaaaaacacccatccaggcagggggatatggagaatttgcagccttcaagtag

SEQ ID NO: 8 - protein, 743 aa, Oryctolagus cuniculus
MGNVWNIKQMIKLTQEHIEALLDKFGGEHNPPSIYLEAYEEYTSKLDALQQREQQLLESLVFQNPTDVSRSNPKSPQKPIVRVFLPNKQRTVVPARCGVTVRDSLKKALMMRGLIPECCAVYRIQDGEKKPIGWDTDISWLTGEELHVEVLENVPLTTHNFVRKTFFTLAFCDFCRKLLFQGFRCQTCGYKFHQRCSTEVPLMCVNYDQLDLLFVSKFFEHHPVPQEEASLAETALTSGSSPSAPPSDSIGHQILTSPSPSKSIPIPQSFRPADEDHRNQFGQRDRSSSAPNVHINTIEPVNIDEKFPEVELQDQRDLIRDQGFRGDGAPLNQLMRCLRKYQSRTPSPLLPSVPSDIVFDFEPGPVFRGSTTGLSATPPASLPGSLTSVKAVQRSPGPQRERKSSSSSEDRNRMKTLGRRDSSDDWEIPDGQITVGQRIGSGSFGTVYKGKWHGDVAVKMLNVTAPTPQQLQAFKNEVGVLRKTRHVNILLFMGYSTKPQLAIVTQWCEGSSLYHHLHIIETKFEMIKLIDIARQTAQGMDYLHAKSIIHRDLKSNNIFLHEDLTVKIGDFGLATVKSRWSGSHQFEQLSGSILWMAPEVIRMQDKNPYSFQSDVYAFGIVLYELMTGQLPYSNINNRDQIIFMVGRGYLSPDLSKVRSNCPKAMKRLMAECLKKKRDERPLFPQILASIELLARSLPKIHRSASEPSLNRAGFQTEDFSLYACASPKTPIQAGGYGEFAAFK

SEQ ID NO: 9 - DNA, 2186 bp, Cavia porcellus
atggcggcgctcagcggcggcggtggcgcggagcagggccaggctctgttcaacggggacatggagctcgaggccggcgccggcgccgcagcctcttcggctgcagaccctgccattcccgaggaggtatggaatatcaaacaaatgattaagttgacgcaggaacacatagaggccctattggacaaatttggtggagagcataatccaccatcaatatacctggaggcctatgaagaatacaccagcaaactagatgccctccaacaaagagaacagcagttactggaatccctcgggaatggaactgatttttctgtttctagctctgcatcactggacaccgttacatcttcttcttcttctagcctttcagtactaccttcatctctttcagtttttcaaaatcctacagatgtgtcacggagcaaccccaaatcaccacaaaaacctattgttagagtcttcctgcccaacaaacagaggacagtggtacctgcaaggtgtggagttacagtccgagacagtctgaagaaagcactcatgatgagaggtcttatcccagagtgctgtgctgtgtacagaattcaggatggagaaaagaaaccaattggctgggacactgacatttcctggcttactggggaagaattacatgtagaagtattggagaatgttccacttacaacacacaattttgtatgtatctttatattttttttgctgtttgtctccaagttctttgaacaccacccaataccacaggaggaggcttccttagcagagaccacccttacatctggatcatccccttctgcacccccctcagagtccattgggcccccaattctcaccagcccatctccttcaaaatccattccaattccacagcctttccggccaggagaggaagatcatcgaaatcaatttgggcagcgagaccggtcctcatctgctcccaatgtgcatataaacacaatagaacctgtcaatattgatgatttgattagagaccaagggtttcgtagtgatggaggatcaactacaggtttgtctgccaccccacctgcctcattacctggctcactcactaatgtgaaagccttacagaaatctccaggacctcagcgagaaaggaagtcatcttcatcctcagaagacagaaatcgaatgaaaacgcttggtagacgggactcaagtgatgattgggagattcctgatgggcagattacagtgggacaaagaattggatctgggtcatttggaacagtctacaaggggaagtggcatggtgacgtggcagtgaaaatgttgaatgtgacagcacccacacctcaacagttacaggccttcaaaaatgaagtaggagtactcaggaaaacacgacatgtgaatatcctactcttcatgggctattccacaaagccacagctagctattgttacccagtggtgtgagggctccagcttataccaccatctccacatcatcgagaccaaatttgagatgatcaaacttatagatattgcacgacagactgcccagggcatggattacttacacgccaagtcaatcatccacagagacctcaagagtaataatatatttcttcacgaagacctcacggttaaaataggtgattttggtctagccacagtgaaatctcgatggagtgggtcccatcagtttgaacagttgtctggatccattttgtggatggcaccagaagtaatcagaatgcgagataaaaacccatacagttttcagtccgatgtatatgcatttgggattgttctatatgaattgatgactgggcagttaccctattcaaatatcaacaacagggaccagataatttttatggtgggacgaggatatctatctccagatctcagcaaggtacggagtaactgtccaaaagccatgaagaggttaatggcggagtgcctcaaaaagaaaagagatgagagaccactctttccccaaattctcgcctctattgagctgctggcccgctcattgccaaaaattcaccgcagtgcatcagaaccctccttgaatcgggctggtttccaaacagaggattttagtctctatgcttgtgcttctccaaaaacacccatccaggcagggggatatggtgcgtttcctgtccactgatgcaaattaaatgagtgagaaataaa

SEQ ID NO: 10 - protein, 719 aa, Cavia porcellus
MAALSGGGGAEQGQALFNGDMELEAGAGAAASSAADPAIPEEVWNIKQMIKLTQEHIEALLDKFGGEHNPPSIYLEAYEEYTSKLDALQQREQQLLESLGNGTDFSVSSSASLDTVTSSSSSSLSVLPSSLSVFQNPTDVSRSNPKSPQKPIVRVFLPNKQRTVVPARCGVTVRDSLKKALMMRGLIPECCAVYRIQDGEKKPIGWDTDISWLTGEELHVEVLENVPLTTHNFVCIFIFFLLFVSKFFEHHPIPQEEASLAETTLTSGSSPSAPPSESIGPPILTSPSPSKSIPIPQPFRPGEEDHRNQFGQRDRSSSAPNVHINTIEPVNIDDLIRDQGFRSDGGSTTGLSATPPASLPGSLTNVKALQKSPGPQRERKSSSSSEDRNRMKTLGRRDSSDDWEIPDGQITVGQRIGSGSFGTVYKGKWHGDVAVKMLNVTAPTPQQLQAFKNEVGVLRKTRHVNILLFMGYSTKPQLAIVTQWCEGSSLYHHLHIIETKFEMIKLIDIARQTAQGMDYLHAKSIIHRDLKSNNIFLHEDLTVKIGDFGLATVKSRWSGSHQFEQLSGSILWMAPEVIRMRDKNPYSFQSDVYAFGIVLYELMTGQLPYSNINNRDQIIFMVGRGYLSPDLSKVRSNCPKAMKRLMAECLKKKRDERPLFPQILASIELLARSLPKIHRSASEPSLNRAGFQTEDFSLYACASPKTPIQAGGYGAFPVH

SEQ ID NO: 11 - DNA, 3229 bp, Canis lupus
gtaatgctggattttcatggaataagtttgacctgtgctgcagtggcctccagcaaggtacccgcaagatgtggagttacagtccgggacagtctaaagaaagctctgatgatgagaggtctaatcccagagtgctgtgctgtttacagaattcaggatggagagaagaaaccgattggctgggacactgatatttcctggctcactggagaggaattgcatgtagaagtgttggaaaatgttccgcttaccacacacaactttgtacggaaaacttttttcaccttagcattttgtgacttttgtcgaaagctgcttttccagggttttcgctgtcaaacatgtggttataaatttcaccagcgttgtagtacagaggttccactgatgtgtgttaattatgaccaacttgatttgctgtttgtctccaagttctttgaacaccacccaataccacaggaggaggcctccatagcagagactgcccttacgtctggatcatccccttctgctcccccctccgattctcctgggcccccaattctgaccagtccgtctccttcaaaatccattccaattccacagcctttccgaccagcagatgaagatcatcgaaatcagtttggacaacgagaccggtcctcatcagctccaaatgtgcatataaacacaatagaacccgtcaacattgatgacttgattagagaccaagggtttcgtagtgatggaggatcaaccacaggtttgtctgccaccccccctgcctcattgcctggctcactcactaatgtaaaagcattacagaaatctccaggacctcagcgggaaagaaaatcatcttcatcctcagaagataggaatcgaatgaaaacacttggtagacgggattcaagtgatgattgggagatacctgatgggcagatcacagtgggacagagaattggatccgggtcatttgggacagtctacaagggaaagtggcatggtgacgtggcagtgaaaatgttgaatgtgacagcacccacacctcagcagttacaggccttcaaaaatgaagtaggagtactcaggaaaactcgacatgtgaatatcctactctttatgggctattcaacaaagccccaactggctattgttacccagtggtgtgagggctccagcttatatcaccatctccacatcattgagaccaaatttgagatgataaagcttatagatattgcacggcagactgcacagggcatggattacttacacgccaagtcaatcatccacagagacctcaagagtaataatatttttcttcatgaagacctcacagtaaaaataggtgattttggtctagccacagtgaaatctcgatggagtgggtcccatcagtttgaacagttgtctggatccattttgtggatggcaccagaagtgatccgaatgcaagacaaaaacccatatagcttccagtcagatgtatacgcatttgggattgttctatatgaattgatgacagggcagttaccttattcaaacatcaacaacagggaccagataatttttatggtgggacgaggatatctttctccagatctcagtaaggtacggagtaactgtccaaaagccatgaagagattgatggcagagtgcctaaaaaagaaaagagatgagaggccactctttccccaaattctcgcctctattgagctgctggcccgctcattgccaaaaattcaccgcagtgcatcagaaccctccttgaatcgggctggcttccaaacagaggattttagtctctatgcttgcgcttctccaaaaacacccatccaggcagggggatacggagaatttgcagccttcaagtagccacaccatcatggcaacaactactcttatttcttaagtcttgtgttcgtacaatttgttaacatcaaaacacagttctgttcctcaaatctttttttaaagatacagaattttcaatgcataagctggtgtggaacagaatggaatttcccatccaacaaaagagggaagaatgttttaggaaccagaattctctgctgccagtgtttcttcttcaacacaaataccacgtgcatacaagtctgcccactcccaggaaggaagaggagagcctgagttctgaccttttgatggtcaggcatgatggaaagaaactgctgctacagcttgggagattggctgtggagagcctgcccgtcagctctgcccttctaaccgccagatgagtgtgtggctggtcacctgacagggcagctgcaatcgccaagcatcgttctctttcctgtcctgggattttgtcgtggagctctttccccctagtcaccaccggttcatttctgagggatggaacaaaaatgcagcatggcctttctgtgtggtgcatgtccggtctttgacaaatttttatcaagtgaagctcttgtatttaaatggagaatgagaggcgagggggggggatcacgttttggtgtaggggcaaagggaatgctgcatctttttcctgacccactgggtttctggcctttgtttccttgctcactgagggtgtctgcctataaccacgcaggctggaaagtgctggcacacattgccttctcttctcactgggtccagcaatgaagacaagtgttggggatttttttttttgccctccacaatgtagcaagttctcaggaaaatacagttaatatcttcctcctaagctcttccagtcatcaagtacttatgtggctactttgtccagggcacaaaatgccatggcggtatccaattaaaagcctacaaaactgcttgataacagttttgaatgtgtgagacatttatgtaatttaaatgtaaggtacaagttttaatttctgagtttctctattatatttttattaaaaagaaaataattttcagatttaattgaattggaataaaataatacttcccaccagaattatatatcctggaaaattgtatttttgttatataaacaacttttaaagaaagatcattatccttttctctacctaaatatggggagtcttagcataatgacagatatttataatttttaaattaatggtacttgctggatccacactaacatctttgctaatatctcatgttttcctccaacttactcctacactacatcctccatcctctttccagtcttttatctagaatatgcaacctaaaataaaaatggtggtgtctccattca

SEQ ID NO: 12 - protein, 617 aa, Canis lupus
MLDFHGISLTCAAVASSKVPARCGVTVRDSLKKALMMRGLIPECCAVYRIQDGEKKPIGWDTDISWLTGEELHVEVLENVPLTTHNFVRKTFFTLAFCDFCRKLLFQGFRCQTCGYKFHQRCSTEVPLMCVNYDQLDLLFVSKFFEHHPIPQEEASIAETALTSGSSPSAPPSDSPGPPILTSPSPSKSIPIPQPFRPADEDHRNQFGQRDRSSSAPNVHINTIEPVNIDDLIRDQGFRSDGGSTTGLSATPPASLPGSLTNVKALQKSPGPQRERKSSSSSEDRNRMKTLGRRDSSDDWEIPDGQITVGQRIGSGSFGTVYKGKWHGDVAVKMLNVTAPTPQQLQAFKNEVGVLRKTRHVNILLFMGYSTKPQLAIVTQWCEGSSLYHHLHIIETKFEMIKLIDIARQTAQGMDYLHAKSIIHRDLKSNNIFLHEDLTVKIGDFGLATVKSRWSGSHQFEQLSGSILWMAPEVIRMQDKNPYSFQSDVYAFGIVLYELMTGQLPYSNINNRDQIIFMVGRGYLSPDLSKVRSNCPKAMKRLMAECLKKKRDERPLFPQILASIELLARSLPKIHRSASEPSLNRAGFQTEDFSLYACASPKTPIQAGGYGEFAAFK

SEQ ID NO: 13 - DNA, 1889 bp, Canis lupus
ggaatatcaaacaaatgattaagttgacacaggaacatatagaagccctattggacaagtttggtggggagcataatccaccatcaatatatctggaggcctatgaagaatacaccagcaaactagatgccctccaacagcgagaacaacagttattggaatccctggggaatggaactgatttttctgtttctagctctgcatcaacggacaccgttacatcttcttcctcttctagcctttcagtgctaccttcatctctttcagtttttcaaaatcccacagatatatcacggagcaatcccaagtcaccacaaaaacctatcgttagagtcttcctgcccaataaacagaggacggtggtacccgcaagatgtggagttacagtccgggacagtctaaagaaagctctgatgatgagaggtctaatcccagagtgctgtgctgtttacagaattcaggatggagagaagaaaccgattggctgggacactgatatttcctggctcactggagaggaattgcatgtagaagtgttggaaaatgttccgcttaccacacacaactttgtacggaaaacttttttcaccttagcattttgtgacttttgtcgaaagctgcttttccagggttttcgctgtcaaacatgtggttataaatttcaccagcgttgtagtacagaggttccactgatgtgtgttaattatgaccaacttgatttgctgtttgtctccaagttctttgaacaccacccaataccacaggaggaggcctccatagcagagactgcccttacgtctggatcatccccttctgctcccccctccgattctcctgggcccccaattctgaccagtccgtctccttcaaaatccattccaattccacagcctttccgaccagcagatgaagatcatcgaaatcagtttggacaacgagaccggtcctcatcagctccaaatgtgcatataaacacaatagaacccgtcaacattgatgacttgattagagaccaagggtttcgtagtgatggaggatcaaccacaggtttgtctgccaccccccctgcctcattgcctggctcactcactaatgtaaaagcattacagaaatctccaggacctcagcgggaaagaaaatcatcttcatcctcagaagataggaatcgaatgaaaacacttggtagacgggattcaagtgatgattgggagatacctgatgggcagatcacagtgggacagagaattggatccgggtcatttgggacagtctacaagggaaagtggcatggtgacgtggcagtgaaaatgttgaatgtgacagcacccacacctcagcagttacaggccttcaaaaatgaagtaggagtactcaggaaaactcgacatgtgaatatcctactctttatgggctattcaacaaagccccaactggctattgttacccagtggtgtgagggctccagcttatatcaccatctccacatcattgagaccaaatttgagatgataaagcttatagatattgcacggcagactgcacagggcatggattacttacacgccaagtcaatcatccacagagacctcaagagtaataatatttttcttcatgaagacctcacagtaaaaataggtgattttggtctagccacagtgaaatctcgatggagtgggtcccatcagtttgaacagttgtctggatccattttgtggatggcaccagaagtgatccgaatgcaagacaaaaacccatatagcttccagtcagatgtatacgcatttgggattgttctatatgaattgatgacagggcagttaccttattcaaacatcaacaacagggaccagctcagatcatgatcacggtgtcatgagatcaagccccac

SEQ ID NO: 14 - protein, 615 aa, Canis lupus
MIKLTQEHIEALLDKFGGEHNPPSIYLEAYEEYTSKLDALQQREQQLLESLGNGTDFSVSSSASTDTVTSSSSSSLSVLPSSLSVFQNPTDISRSNPKSPQKPIVRVFLPNKQRTVVPARCGVTVRDSLKKALMMRGLIPECCAVYRIQDGEKKPIGWDTDISWLTGEELHVEVLENVPLTTHNFVRKTFFTLAFCDFCRKLLFQGFRCQTCGYKFHQRCSTEVPLMCVNYDQLDLLFVSKFFEHHPIPQEEASIAETALTSGSSPSAPPSDSPGPPILTSPSPSKSIPIPQPFRPADEDHRNQFGQRDRSSSAPNVHINTIEPVNIDDLIRDQGFRSDGGSTTGLSATPPASLPGSLTNVKALQKSPGPQRERKSSSSSEDRNRMKTLGRRDSSDDWEIPDGQITVGQRIGSGSFGTVYKGKWHGDVAVKMLNVTAPTPQQLQAFKNEVGVLRKTRHVNILLFMGYSTKPQLAIVTQWCEGSSLYHHLHIIETKFEMIKLIDIARQTAQGMDYLHAKSIIHRDLKSNNIFLHEDLTVKIGDFGLATVKSRWSGSHQFEQLSGSILWMAPEVIRMQDKNPYSFQSDVYAFGIVLYELMTGQLPYSNINNRDQLRS

SEQ ID NO: 15 - DNA, 3521 bp, Felis catus
  misc_feature (630)..(649): n is a, c, g, or t
atgcctaacctcagtctctgccaccacggccaatttgctcatgtgcccactgtgtcggcactgggatattttgtgatttgccttggccattgtccactgtccttgacattgcctgaaggagaaccactgatgctaatgttgaaggtgacctttgcaggctctccactactcataccaaagatgcggccccctgataatcccagagccactgtctgcacatgggcaaaacaggctacattctgtgcagactggggagaaaggttccaagaacacagtgccatagttttgggcagagagtttcaacacagcatagtgtctatggcagtatctggatttggccgggggaagtgcccaagaggagacagtcaggctgtgtcctacggccaaggacctgcacttatttttgcatgcagtggtttagcacagggaagagaacgaagtaggaaatcggagccatggaaacggcagagcggaggaaacgtgcacgcgcgagggtgggcacgaaaggaaagaaccctccccagaagactgcgcgagggcgctcctaggattacgtcacgcaccccgcgaaaactgaaatgtactgtgtgtggtcttttaattgaactatcttccttatgtgcacttaannnnnnnnnnnnnnnnnnnngcggcggcggcggtggcgcggagcagggccaggctctgttcaacggggacatggagcccgaagccggcgccgcggcctcttcggctgcggaccctgccattcccgaggaggtgtggaatatcaaacaaatgattaagttgacacaggaacatatagaggccctattggacaaatttggtggggagcataatccaccatcaatatatctagaggcctatgaagaatacaccagcaagctagatgccctccaacagagagaacaacagttattggaatccctggggaatggaactgatttttctgtttctagctctgcatcaacagacaccgttacatcttcctcctcttctagcctttcagtgctaccttcatctctttcagtttttcaaaaccccacagatgtgtcacggagcaatcccaagtcaccacagaaacctatcgttagagtcttcctgcctaataaacagaggacagtggtacctgcaagatgtggagttacagtccgggacagtctaaagaaagctctgatgatgagaggtctaatccctgagtgctgtgctgtttacagaattcaggatggagagaagaaaccaattggctgggacactgatatctcctggctcaccggagaggaattgcatgtagaagtgttggaaaatgttccacttacaactcacaactttgtatgtacggaaaacgttttcaccttagcattttgtgacttttgtcgaaagctgcttttccaaggttttcgctgtcaaacgtgtggttataaatttcaccagcgttgtagtacagaggttccactgatgtgtgttaattatgaccaacttgatttgctgtttgtctccaagttctttgaacaccacccaataccacaggaggaggcctccatagcagagactgccctaacgtctggatcgtccccttctgcccccccctccgattctactgggccccaaattctcaccagtccgtctccttcaaaatccattccaattccacagcctttccgaccagcagatgaagatcatcgaaatcaatttggacagcgagaccggtcctcatcagctccaaatgtgcatataaatacaatagaacctgtcaatattgatgacttgattagagaccaggggtttcgtagtgatggaggatcaaccacaggcttgtctgccaccccccctgcctcattgccgggctctctcactaatgtaaaagcattacagaaatctccagggcctcagcgggaaaggaaatcttcttcatcctcagaagataggaatcgaatgaaaacacttggtagaagggattcaagtgatgattgggagattcctgatgggcagatcacagtgggacagagaattggatccgggtcatttgggacagtctacaagggaaagtggcatggtgatgtggcagtgaaaatgttgaatgtgacagcacccacacctcagcagttacaggccttcaaaaatgaagtaggagtactcaggaaaactcggcatgtgaacatcctgctcttcatgggctattcaacaaagccccagctggctattgtcacccagtggtgtgagggctccagcttataccaccatctccacatcatcgagaccaaattcgagatgatcaagctgatagatattgctcggcagactgcgcagggcatggattacttacacgccaagtcaatcatccacagagacctcaagagtaataatatttttcttcacgaagacctcacagtaaaaataggtgattttggtctagccacagtgaaatctcgatggagtgggtcccatcagtttgaacagttgtctggatccattttgtggatggcaccagaagtaattcgaatgcaagataaaaacccatatagctttcagtcagatgtatatgcatttgggattgttctatatgaattgatgactggacagttaccttattcaaacatcaacaacagggaccagataatttttatggtgggacgaggatatctttctccagatctcagtaaggtacgaagtaactgtccaaaagccatgaagagattgatggcagagtgcctaaaaaagaaaagagatgagaggccactgtttccccaaattcttgcctctattgagctgctggcccgctcattgccaaaaattcaccgcagtgcatcagaaccctccttgaatcgggctggcttccagacagaggattttagtctctatgcttgtgcttctccaaaaacacccatccaggcagggggatatggtgcgtttcccgtccactgagataagttagatgagtgcgcgagtgcagggggccggggccaaggaggtggaaatgtgcgtgcttctgtactaagttggatagcatcttcttttttaaaaaaagatgaaccaaagaatgtgtatgtttttaaagactagatataattatttcctgatctaaaatgtatacttagctttggattttcaatatccaagggttttcaaaatgcacagacattgctgaacatttgcagtacctcttctggaggctttacttcctgttacaaattggttttgtttactggcttatcctaattattaaacttcaattaaacttttctcctgcaccttttgttatgagctatcacatgtcccttagggactcgcaagagcagtactgcccccgtgtacgggcttgcaggtagaaaggggatgacgggttttaacacctgtgtgaggcaaggcagtccgaacagatctcatttaggaagccacgagagttgaataagttatttttattcttagtattttttctgtaactactttttattataacttggaaaatatggatgtcctttatacaccttagcaatagactgaatttctttttataaatt

SEQ ID NO: 16 - protein, 974 aa, Felis catus
  misc_feature (210)..(217): Xaa can be any naturally occurring amino acid
MPNLSLCHHGQFAHVPTVSALGYFVICLGHCPLSLTLPEGEPLMLMLKVTFAGSPLLIPKMRPPDNPRATVCTWAKQATFCADWGERFQEHSAIVLGREFQHSIVSMAVSGFGRGKCPRGDSQAVSYGQGPALIFACSGLAQGRERSRKSEPWKRQSGGNVHARGWARKERTLPRRLREGAPRITSRTPRKLKCTVCGLLIELSSLCALXXXXXXXXGGGGGAEQGQALFNGDMEPEAGAAASSAADPAIPEEVWNIKQMIKLTQEHIEALLDKFGGEHNPPSIYLEAYEEYTSKLDALQQREQQLLESLGNGTDFSVSSSASTDTVTSSSSSSLSVLPSSLSVFQNPTDVSRSNPKSPQKPIVRVFLPNKQRTVVPARCGVTVRDSLKKALMMRGLIPECCAVYRIQDGEKKPIGWDTDISWLTGEELHVEVLENVPLTTHNFVCTENVFTLAFCDFCRKLLFQGFRCQTCGYKFHQRCSTEVPLMCVNYDQLDLLFVSKFFEHHPIPQEEASIAETALTSGSSPSAPPSDSTGPQILTSPSPSKSIPIPQPFRPADEDHRNQFGQRDRSSSAPNVHINTIEPVNIDDLIRDQGFRSDGGSTTGLSATPPASLPGSLTNVKALQKSPGPQRERKSSSSSEDRNRMKTLGRRDSSDDWEIPDGQITVGQRIGSGSFGTVYKGKWHGDVAVKMLNVTAPTPQQLQAFKNEVGVLRKTRHVNILLFMGYSTKPQLAIVTQWCEGSSLYHHLHIIETKFEMIKLIDIARQTAQGMDYLHAKSIIHRDLKSNNIFLHEDLTVKIGDFGLATVKSRWSGSHQFEQLSGSILWMAPEVIRMQDKNPYSFQSDVYAFGIVLYELMTGQLPYSNINNRDQIIFMVGRGYLSPDLSKVRSNCPKAMKRLMAECLKKKRDERPLFPQILASIELLARSLPKIHRSASEPSLNRAGFQTEDFSLYACASPKTPIQAGGYGAFPVH

SEQ ID NO: 17 - DNA, 3853 bp, Bos taurus
ctcagctgcgccgggtctcacaagacggttcccgaggtggcccaggcgccgtcccaccgccgacgccgcccgggccgcccgggccgtccctccccgctgccccccgtcctccgcctccgcctccccccgccctcagcctcccttccccctccccgcccagcagcggtcgctcgggcccggctctcggttataagatggcggcgctgagtggcggcggcggcggcggcggcggtggcgcggagcagggccaggctctgttcaacggggacatggagcccgaggccggcgccgcggcctcttcggctgcggaccccgccattcccgaggaggtgtggaatatcaaacaaatgattaagttgacacaggagcatatagaggccctattggacaaatttggtggggagcataatccaccatcaatatatctggaggcctatgaagaatacaccagcaagctagatgccctccaacaaagagaacaacagttattggaatccctggggaatggaactgatttttctgtttctagctctgcatcaacggacaccgttacatcttcttcctcttctagcctttcagtgctgccttcatctctttcagtttttcaaaatcccacagatgtgtcacggagcaaccccaagtcaccacaaaaacctatcgttagagtcttcctgcccaataaacagaggacagtggtacctgcacggtgtggagtcacagtccgggacagcctgaagaaggcactgatgatgagaggtctaatcccagagtgctgtgctgtttacagaattcaggatggggagaagaaaccaattggctgggacactgatatttcctggcttactggagaggagttgcatgtagaagtgttggagaatgttccacttacaacacacaactttgtacggaaaacttttttcaccttagcattttgtgacttctgtagaaagctgcttttccagggattccgctgtcaaacatgtggttataaatttcaccagcgttgtagtacagaggttccactgatgtgtgttaattatgaccaactagatttgctgtttgtctccaagttctttgaacaccacccaataccacaggaggaggcctccttagcagagactacccttccatgtggctcatccccttctgcacccccctccgattctattgggcccccaattctcaccagtccatctccttcaaaatccattccaattccacagcctttccgaccagcagatgaagatcatcgaaatcagtttggacaacgagaccggtcctcatcagctccaaatgtgcatataaacacaatagaacccgtcaatattgatgacttgattagagaccaagggtttcgtagtgatggaggatcaaccacaggtttatccgccacaccccctgcctcattacctggctcactctctaatgtgaaagcattgcagaaatctccaggacctcagcgagaaagaaagtcctcttcatcctcagaagacaggaatcgaatgaaaacgcttggtagacgggattcaagtgacgattgggagattcctgatggacagatcacagtgggacaaagaattggatcagggtcatttgggacagtctacaagggaaagtggcatggtgatgtggcagtgaaaatgttgaatgtgacagcacccacacctcagcagttacaggccttcaaaaatgaagtaggagtactcaggaaaacgcgacatgtgaatatcctcctcttcatgggttattcaacaaagccacaactggctattgttacccagtggtgtgagggctccagtttatatcatcatctccacatcattgagaccaaattcgagatgatcaaacttatagatattgcacggcagactgcacagggcatggattacttacacgccaagtcaatcatccacagagacctcaagagtaataatatttttcttcatgaagacctcacagtaaaaataggtgattttggtctagccacagtgaaatctcgatggagtgggtcccatcagtttgaacagttgtctggatccattttgtggatggcaccagaagtaatcagaatgcaagataaaaacccatatagctttcagtcagatgtatatgcatttgggattgttctgtatgaattgatgaccggacagttaccttattcaaatatcaacaacagggaccagataatttttatggtgggacgaggatatctgtctccagatctcagtaaggtacggagtaactgtccaaaagccatgaagagattaatggcagagtgcctaaaaaagaaaagagatgaaagaccactctttccccaaattctcgcctctattgagctgctggcccgctcattgccaaaaattcaccgcagtgcatcagaaccctccttgaatcgggctggcttccaaacagaggattttagtctatatgcttgtgcttctccaaaaacacccattcaggcagggggatatggtacgtttcctgttcactgaaacaaaccgagtgagtgacagcatgtaggagggtagggacaaaagaaagtgaacaaatgtttgcttatatatttgttaaattgaataggattttctttttctttaaaggtgaacaagagaacatgtgtgtttttaaagtttggatatagttttcttcccagtctaaaacccatagttagcattacattttcaacatcgaatttttttttaattcatagacattgctgaaaatttataataccttttccagaggctttacttcccattccaagtttgttttgtttacttggttagtctaatcattaaactttaaactttccccacctaccttttgctgttagctatcccgcatccattaggggctccaagaacagcactgtctgcgtgtgtgtgttggcaggtgggaagctgatggtaagttaggctgtgttagtgaaggtaaactgaccaggtctaattaggagtcactagaattgaataagcttatttttattaatattttttcttataactatttctttttgtaataatttagaaaatataattgttctttattcccttacagcagtataaattattggtgcaggtaaccaaagatattactgaggagtggcatgtttgacatgagtgacatggtttaactttggatttttagttaatatttctttatatattaaggatgtcttacacattatagaagtcaaatttactgacaaaggtattgcctcctcttcctccccaaaaacacagcaaaattctctgggaactcgtagcattgttggttttcttttggatgactatggttgccaaacaaccaagtaattgattttttttaaattattattgctttagattatactcacctctcatgatgcctgttagcaatcacctttatccatgtgtcttgtaaaatatctttcctccttatattctttgcccaacaagagtctacttgttatgaatgagtactattttctttttttgattccccagtataattagtatgtttagtgctttctaggacttccactttcttatgttaaaaaaaaaaacaaactaatgtggcagtcagtatattcttactgtgaatcagagtctttactgggaatcaaagtgaaagaagcagctgttctgacttcagagtcagcctagggaccaaaaccagcctcttaaatacaccttcatttattcagtttggatttgtgatgattttcattatagctgacagttcaaggttattcagtggcacacagatagcatctgcataaatgcctttcttcttgaaaataaaggagaaaattgggaagactttacaccaatagtttagtctttaagtaccacagataacacacaccataaat

SEQ ID NO: 18 - protein, 764 aa, Bos taurus
AALSGGGGGGGGGAEQGQALFNGDMEPEAGAAASSAADPAIPEEVWNIKQMIKLTQEHIEALLDKFGGEHNPPSIYLEAYEEYTSKLDALQQREQQLLESLGNGTDFSVSSSASTDTVTSSSSSSLSVLPSSLSVFQNPTDVSRSNPKSPQKPIVRVFLPNKQRTVVPARCGVTVRDSLKKALMMRGLIPECCAVYRIQDGEKKPIGWDTDISWLTGEELHVEVLENVPLTTHNFVRKTFFTLAFCDFCRKLLFQGFRCQTCGYKFHQRCSTEVPLMCVNYDQLDLLFVSKFFEHHPIPQEEASLAETTLPCGSSPSAPPSDSIGPPILTSPSPSKSIPIPQPFRPADEDHRNQFGQRDRSSSAPNVHINTIEPVNIDDLIRDQGFRSDGGSTTGLSATPPASLPGSLSNVKALQKSPGPQRERKSSSSSEDRNRMKTLGRRDSSDDWEIPDGQITVGQRIGSGSFGTVYKGKWHGDVAVKMLNVTAPTPQQLQAFKNEVGVLRKTRHVNILLFMGYSTKPQLAIVTQWCEGSSLYHHLHIIETKFEMIKLIDIARQTAQGMDYLHAKSIIHRDLKSNNIFLHEDLTVKIGDFGLATVKSRWSGSHQFEQLSGSILWMAPEVIRMQDKNPYSFQSDVYAFGIVLYELMTGQLPYSNINNRDQIIFMVGRGYLSPDLSKVRSNCPKAMKRLMAECLKKKRDERPLFPQILASIELLARSLPKIHRSASEPSLNRAGFQTEDFSLYACASPKTPIQAGGYGTFPVH

SEQ ID NO: 19 - DNA, 4936 bp, Bos taurus
ctcagctgcgccgggtctcacaagacggttcccgaggtggcccaggcgccgtcccaccgccgacgccgcccgggccgcccgggccgtccctccccgctgccccccgtcctccgcctccgcctccccccgccctcagcctcccttccccctccccgcccagcagcggtcgctcgggcccggctctcggttataagatggcggcgctgagtggcggcggcggcggcggcggcggtggcgcggagcagggccaggctctgttcaacggggacatggagcccgaggccggcgccgcggcctcttcggctgcggaccccgccattcccgaggaggtgtggaatatcaaacaaatgattaagttgacacaggagcatatagaggccctattggacaaatttggtggggagcataatccaccatcaatatatctggaggcctatgaagaatacaccagcaagctagatgccctccaacaaagagaacaacagttattggaatccctggggaatggaactgatttttctgtttctagctctgcatcaacggacaccgttacatcttcttcctcttctagcctttcagtgctgccttcatctctttcagtttttcaaaatcccacagatgtgtcacggagcaaccccaagtcaccacaaaaacctatcgttagagtcttcctgcccaataaacagaggacagtggtacctgcacggtgtggagtcacagtccgggacagcctgaagaaggcactgatgatgagaggtctaatcccagagtgctgtgctgtttacagaattcaggatggggagaagaaaccaattggctgggacactgatatttcctggcttactggagaggagttgcatgtagaagtgttggagaatgttccacttacaacacacaactttgtacggaaaacttttttcaccttagcattttgtgacttctgtagaaagctgcttttccagggattccgctgtcaaacatgtggttataaatttcaccagcgttgtagtacagaggttccactgatgtgtgttaattatgaccaactagatttgctgtttgtctccaagttctttgaacaccacccaataccacaggaggaggcctccttagcagagactacccttccatgtggctcatccccttctgcacccccctccgattctattgggcccccaattctcaccagtccatctccttcaaaatccattccaattccacagcctttccgaccagcagatgaagatcatcgaaatcagtttggacaacgagaccggtcctcatcagctccaaatgtgcatataaacacaatagaacccgtcaatattgatgacttgattagagaccaagggtttcgtagtgatggaggatcaaccacaggtttatccgccacaccccctgcctcattacctggctcactctctaatgtgaaagcattgcagaaatctccaggacctcagcgagaaagaaagtcctcttcatcctcagaagacaggaatcgaatgaaaacgcttggtagacgggattcaagtgacgattgggagattcctgatggacagatcacagtgggacaaagaattggatcagggtcatttgggacagtctacaagggaaagtggcatggtgatgtggcagtgaaaatgttgaatgtgacagcacccacacctcagcagttacaggccttcaaaaatgaagtaggagtactcaggaaaacgcgacatgtgaatatcctcctcttcatgggttattcaacaaagccacaactggctattgttacccagtggtgtgagggctccagtttatatcatcatctccacatcattgagaccaaattcgagatgatcaaacttatagatattgcacggcagactgcacagggcatggattacttacacgccaagtcaatcatccacagagacctcaagagtaataatatttttcttcatgaagacctcacagtaaaaataggtgattttggtctagccacagtgaaatctcgatggagtgggtcccatcagtttgaacagttgtctggatccattttgtggatggcaccagaagtaatcagaatgcaagataaaaacccatatagctttcagtcagatgtatatgcatttgggattgttctgtatgaattgatgaccggacagttaccttattcaaatatcaacaacagggaccagataatttttatggtgggacgaggatatctgtctccagatctcagtaaggtacggagtaactgtccaaaagccatgaagagattaatggcagagtgcctaaaaaagaaaagagatgaaagaccactctttccccaagtaggaaagactctcctaagcaagagacaaaattcagaagttatcagggaaaaagataagcagattctcgcctctattgagctgctggcccgctcattgccaaaaattcaccgcagtgcatcagaaccctccttgaatcgggctggcttccaaacagaggattttagtctatatgcttgtgcttctccaaaaacacccattcaggcagggggatatgaagcagatttggctcttacatcaaataaaaatagagtagaagttgggatttagagatttcctgacatgcaagaaggaataagcaagaaaaaaaggtttgttttccccaaatcatatctattgtcttttacttctattttttcttaaattttttgtgatttcagagacatgtagagttttattgatacctaaactatgagttcttttttttttttttttttcattattttgatttttttggccaagaggcatatgggatcttagcttgagaaagcaacaattttcttgatgtcattttgggtgagggcacatattgctgtgaacagtgtggtgatagccaccagggaccaaactcacacccgctgcattgaaaggtgaagtcttaaacactggaccagcagagaaattcctactctatgagttctttttgtcatcccctccccgcaccctccacccccaacctaaagtctgatgatgaaatcaacaactattccattagaagcagtagattctggtagcatgatctttagtttgttagtaagattttgtgctttgtggggttgtgtcgttttaaggctaatatttaagtttgtcaaatagaatgctgttcagattgtaaaaatgagtaataaacatctgaagttttttttaagttatttttaacatggtatatacagttgagcttagagtttatcattttctgatattctcttacttagtagatgaattctagccattttttataaagatttctgttaagcaaatcctgttttcacatgggcttcctttaagggattttagattctgctggatatggtgactgctcataagactgttgaaaattacttttaagatgtattagaatacttctgaaaaaaaatagcaaccttaaaaccataagcaaaagtagtaagggtgtttatacatttctagagtccctgtttaggtaatagcctcctatgattgtactttaaatgttttgctctccaaggttttagtaacttggctttttttctaatcagtgccaaactcccccagtttttttaactttaaatatgaggtaataaatcttttacccttccttgatcttttgacttataataccttggtcagttgtttcttaaaaggaatccttaaatggaaagagacaatatcactgtctgcagttctgattagtagttttattcagaatggaaaaacagattattcatttttgaaaattgttcaggggtatgttcattgttaggaccttggactttggagtcagtgcctagctatgcattccaggtctgccattttctggctgtgaaattttggacaagttacttaaccactttaaaccccagctttaagaagtaaattaaccccagtaaattaagaagtaatagcagccacttcgtagagttgttatgaggctcagatgcagtgcaaatgtgtataaagtattcagggagtcacctggtatactataatagacactagaatagttgccaatattatcagcatacaatctgaggattctgtcagccaatcattagcaatctgttgtttgttgggacatgccagtgttctccagttgaaatcagtagcaatctaaaaatggatagattattcctcatttaaatagtgtgttcatataagtgattgcttggatccttatcagaagttgctgttactgaaaaatgataaggctgactaaattgtgatagttgtcagttactaaccaactcccagaaatgaataagaggaacctatctctagttcctagtagaaggtatggacaaaatagtaggtgaaaaataatgtcttgaacccccaaattaagtaagctttaaagagtacaatacctcaaagggtctttgcggtttaaaatttgtatgctgagaatgatgttcattgacatgtgcctatatgtaattttttgatagtttaaaaggtgaaatgaactacagatgggagaggtctgaattttcttgccttcagtcaaatgtgtaatgtggacatattatttgacctgtgaattttatcttttaaaaaagattaattcctgcttcttccttcctaatagttgcattataataatgaaaatgagttgataatttggggggaaagtattctacaaatcaaccttattattttaccattggtttctgagaaattttgttcatttgaaccgtttatagcttgattagaatcatagcatgtaaaacccaactgagggattatctgcagacttaatgtagtattatgtaagttgtcttctttcatttcgaccttttttgcttttgttgttgctagatctgtagtatgtagctagtcacctttcagcgaggtttcagcgaggcttttctgtgtctctaggttatttgagataacttttttaaaattagctcttgtcctcc

SEQ ID NO: 20 - protein, 797 aa, Bos taurus
MAALSGGGGGGGGGAEQGQALFNGDMEPEAGAAASSAADPAIPEEVWNIKQMIKLTQEHIEALLDKFGGEHNPPSIYLEAYEEYTSKLDALQQREQQLLESLGNGTDFSVSSSASTDTVTSSSSSSLSVLPSSLSVFQNPTDVSRSNPKSPQKPIVRVFLPNKQRTVVPARCGVTVRDSLKKALMMRGLIPECCAVYRIQDGEKKPIGWDTDISWLTGEELHVEVLENVPLTTHNFVRKTFFTLAFCDFCRKLLFQGFRCQTCGYKFHQRCSTEVPLMCVNYDQLDLLFVSKFFEHHPIPQEEASLAETTLPCGSSPSAPPSDSIGPPILTSPSPSKSIPIPQPFRPADEDHRNQFGQRDRSSSAPNVHINTIEPVNIDDLIRDQGFRSDGGSTTGLSATPPASLPGSLSNVKALQKSPGPQRERKSSSSSEDRNRMKTLGRRDSSDDWEIPDGQITVGQRIGSGSFGTVYKGKWHGDVAVKMLNVTAPTPQQLQAFKNEVGVLRKTRHVNILLFMGYSTKPQLAIVTQWCEGSSLYHHLHIIETKFEMIKLIDIARQTAQGMDYLHAKSIIHRDLKSNNIFLHEDLTVKIGDFGLATVKSRWSGSHQFEQLSGSILWMAPEVIRMQDKNPYSFQSDVYAFGIVLYELMTGQLPYSNINNRDQIIFMVGRGYLSPDLSKVRSNCPKAMKRLMAECLKKKRDERPLFPQVGKTLLSKRQNSEVIREKDKQILASIELLARSLPKIHRSASEPSLNRAGFQTEDFSLYACASPKTPIQAGGYEADLALTSNKNRVEVGI

SEQ ID NO: 21 - DNA, 4154 bp, Bos taurus
ctcagctgcgccgggtctcacaagacggttcccgaggtggcccaggcgccgtcccaccgccgacgccgcccgggccgcccgggccgtccctccccgctgccccccgtcctccgcctccgcctccccccgccctcagcctcccttccccctccccgcccagcagcggtcgctcgggcccggctctcggttataagatggcggcgctgagtggcggcggcggcggcggcggcggtggcgcggagcagggccaggctctgttcaacggggacatggagcccgaggccggcgccgcggcctcttcggctgcggaccccgccattcccgaggaggtgtggaatatcaaacaaatgattaagttgacacaggagcatatagaggccctattggacaaatttggtggggagcataatccaccatcaatatatctggaggcctatgaagaatacaccagcaagctagatgccctccaacaaagagaacaacagttattggaatccctggggaatggaactgatttttctgtttctagctctgcatcaacggacaccgttacatcttcttcctcttctagcctttcagtgctgccttcatctctttcagtttttcaaaatcccacagatgtgtcacggagcaaccccaagtcaccacaaaaacctatcgttagagtcttcctgcccaataaacagaggacagtggtacctgcacggtgtggagtcacagtccgggacagcctgaagaaggcactgatgatgagaggtctaatcccagagtgctgtgctgtttacagaattcaggatggggagaagaaaccaattggctgggacactgatatttcctggcttactggagaggagttgcatgtagaagtgttggagaatgttccacttacaacacacaactttgtacggaaaacttttttcaccttagcattttgtgacttctgtagaaagctgcttttccagggattccgctgtcaaacatgtggttataaatttcaccagcgttgtagtacagaggttccactgatgtgtgttaattatgaccaactagatttgctgtttgtctccaagttctttgaacaccacccaataccacaggaggaggcctccttagcagagactacccttccatgtggctcatccccttctgcacccccctccgattctattgggcccccaattctcaccagtccatctccttcaaaatccattccaattccacagcctttccgaccagcagatgaagatcatcgaaatcagtttggacaacgagaccggtcctcatcagctccaaatgtgcatataaacacaatagaacccgtcaatattgatgacttgattagagaccaagggtttcgtagtgatggaggatcaaccacaggtttatccgccacaccccctgcctcattacctggctcactctctaatgtgaaagcattgcagaaatctccaggacctcagcgagaaagaaagtcctcttcatcctcagaagacaggaatcgaatgaaaacgcttggtagacgggattcaagtgacgattgggagattcctgatggacagatcacagtgggacaaagaattggatcagggtcatttgggacagtctacaagggaaagtggcatggtgatgtggcagtgaaaatgttgaatgtgacagcacccacacctcagcagttacaggccttcaaaaatgaagtaggagtactcaggaaaacgcgacatgtgaatatcctcctcttcatgggttattcaacaaagccacaactggctattgttacccagtggtgtgagggctccagtttatatcatcatctccacatcattgagaccaaattcgagatgatcaaacttatagatattgcacggcagactgcacagggcatggattacttacacgccaagtcaatcatccacagagacctcaagagtaataatatttttcttcatgaagacctcacagtaaaaataggtgattttggtctagccacagtgaaatctcgatggagtgggtcccatcagtttgaacagttgtctggatccattttgtggatggcaccagaagtaatcagaatgcaagataaaaacccatatagctttcagtcagatgtatatgcatttgggattgttctgtatgaattgatgaccggacagttaccttattcaaatatcaacaacagggaccagataatttttatggtgggacgaggatatctgtctccagatctcagtaaggtacggagtaactgtccaaaagccatgaagagattaatggcagagtgcctaaaaaagaaaagagatgaaagaccactctttccccaagtaggaaagactctcctaagcaagagacaaaattcagaagttatcagggaaaaagataagcagattctcgcctctattgagctgctggcccgctcattgccaaaaattcaccgcagtgcatcagaaccctccttgaatcgggctggcttccaaacagaggattttagtctatatgcttgtgcttctccaaaaacacccattcaggcagggggatatggctgagcacattgtccatcacccacaagtggctggttctcatcgcagaatctacgtagggaatcgggcgtgaaattcacttaagagatagagcagaggaagtgttctgtttacaggaatggagatgagagttatgagtaagttgcttagtcagttggctttgttttgaaaattattgtgttatatttgtgttaacctacttgtgttttgacagtatatgtcacataggaagaaacctcagactagcataataacaaagctcagactaggcacagatgtacacagaatggaccaaaatgggatgggggaaggtatgggaataagtctaggggtagggaaaaattgatgtgagggtgggaaataaactgtaattacctgaaataaaatgtaagagtgcaataagtgtgctttttattctaagctgtgaatgggttttttaaaaaaagcattccttcccaatgcatttgcctatgttccatagctgattaaaaccagctatataaacatatgcctttttattcatgttaattaccaatataaatggctaacctttacgtcttatttatcttcatgttatgttagtttacatacagggatgtgtgtgtgtgtgtatgctataaattttccctccttcgtttaaaaacgcgtttgttggatcctctctgtttccttaggccatgccacagctcatagtctcagcttggccttcctgtcacctgatctgaaggactatcacagtgacgtagctcgttcattggttgtacacactctaacccttttccttgctcagcaattactgtgtcttctaaaacaggagtgtacaaccatgagattgcaattaattgtttgacatatgtccctttgaattctatttattagttatgattgattgctctttggtttggaccaagaaaaacgaaatcccacctccccaccttttcacttatttcttactttgaggacaattctgtaagagagaggaaagggaactccttcatgttttaactgcagcaagttaatggccctggtttacaccaaacattatggtgattcacattcacattcctctcctctcttgctgccagaggtttgggttttgttcagttctgctcaagcactgaaaaagttttcatggagtctggagagtgcccagtgaaaagatggtttttaattgtccacagacctttctgttcctgctttgcaaaaattacaaaggagtaactatttttaaagcttatttttcaattcataaaaaagacatttattttcagtcagatgatgtctccttgtcccttaatcctcaatgtttgcttgaatcttttttttttttctgattttctcccatccccacttcttgatacttcttgagttctctttcctgctcaggtcctttcatttgtactttggagttttttctcatgtaaatttgtacaatggaaaatattgttcagtttggatagaacgcatggagaattaaataaaaaagatagctgaaattcagattgaaatttatttgtgtaaagttatttaaaaactctgtactatataaaaggcaaaaaaagttctatgtacttgatgtgaatatgcgaatactgctataataaagattgactgcatgga

SEQ ID NO: 22 - protein, 781 aa, Bos taurus
MAALSGGGGGGGGGAEQGQALFNGDMEPEAGAAASSAADPAIPEEVWNIKQMIKLTQEHIEALLDKFGGEHNPPSIYLEAYEEYTSKLDALQQREQQLLESLGNGTDFSVSSSASTDTVTSSSSSSLSVLPSSLSVFQNPTDVSRSNPKSPQKPIVRVFLPNKQRTVVPARCGVTVRDSLKKALMMRGLIPECCAVYRIQDGEKKPIGWDTDISWLTGEELHVEVLENVPLTTHNFVRKTFFTLAFCDFCRKLLFQGFRCQTCGYKFHQRCSTEVPLMCVNYDQLDLLFVSKFFEHHPIPQEEASLAETTLPCGSSPSAPPSDSIGPPILTSPSPSKSIPIPQPFRPADEDHRNQFGQRDRSSSAPNVHINTIEPVNIDDLIRDQGFRSDGGSTTGLSATPPASLPGSLSNVKALQKSPGPQRERKSSSSSEDRNRMKTLGRRDSSDDWEIPDGQITVGQRIGSGSFGTVYKGKWHGDVAVKMLNVTAPTPQQLQAFKNEVGVLRKTRHVNILLFMGYSTKPQLAIVTQWCEGSSLYHHLHIIETKFEMIKLIDIARQTAQGMDYLHAKSIIHRDLKSNNIFLHEDLTVKIGDFGLATVKSRWSGSHQFEQLSGSILWMAPEVIRMQDKNPYSFQSDVYAFGIVLYELMTGQLPYSNINNRDQIIFMVGRGYLSPDLSKVRSNCPKAMKRLMAECLKKKRDERPLFPQVGKTLLSKRQNSEVIREKDKQILASIELLARSLPKIHRSASEPSLNRAGFQTEDFSLYACASPKTPIQAGGYG

SEQ ID NO: 23 - DNA, 7914 bp, Bos taurus
ctcagctgcgccgggtctcacaagacggttcccgaggtggcccaggcgccgtcccaccgccgacgccgcccgggccgcccgggccgtccctccccgctgccccccgtcctccgcctccgcctccccccgccctcagcctcccttccccctccccgcccagcagcggtcgctcgggcccggctctcggttataagatggcggcgctgagtggcggcggcggcggcggcggcggtggcgcggagcagggccaggctctgttcaacggggacatggagcccgaggccggcgccgcggcctcttcggctgcggaccccgccattcccgaggaggtgtggaatatcaaacaaatgattaagttgacacaggagcatatagaggccctattggacaaatttggtggggagcataatccaccatcaatatatctggaggcctatgaagaatacaccagcaagctagatgccctccaacaaagagaacaacagttattggaatccctggggaatggaactgatttttctgtttctagctctgcatcaacggacaccgttacatcttcttcctcttctagcctttcagtgctgccttcatctctttcagtttttcaaaatcccacagatgtgtcacggagcaaccccaagtcaccacaaaaacctatcgttagagtcttcctgcccaataaacagaggacagtggtacctgcacggtgtggagtcacagtccgggacagcctgaagaaggcactgatgatgagaggtctaatcccagagtgctgtgctgtttacagaattcaggatggggagaagaaaccaattggctgggacactgatatttcctggcttactggagaggagttgcatgtagaagtgttggagaatgttccacttacaacacacaactttgtacggaaaacttttttcaccttagcattttgtgacttctgtagaaagctgcttttccagggattccgctgtcaaacatgtggttataaatttcaccagcgttgtagtacagaggttccactgatgtgtgttaattatgaccaactagatttgctgtttgtctccaagttctttgaacaccacccaataccacaggaggaggcctccttagcagagactacccttccatgtggctcatccccttctgcacccccctccgattctattgggcccccaattctcaccagtccatctccttcaaaatccattccaattccacagcctttccgaccagcagatgaagatcatcgaaatcagtttggacaacgagaccggtcctcatcagctccaaatgtgcatataaacacaatagaacccgtcaatattgatgacttgattagagaccaagggtttcgtagtgatggaggatcaaccacaggtttatccgccacaccccctgcctcattacctggctcactctctaatgtgaaagcattgcagaaatctccaggacctcagcgagaaagaaagtcctcttcatcctcagaagacaggaatcgaatgaaaacgcttggtagacgggattcaagtgacgattgggagattcctgatggacagatcacagtgggacaaagaattggatcagggtcatttgggacagtctacaagggaaagtggcatggtgatgtggcagtgaaaatgttgaatgtgacagcacccacacctcagcagttacaggccttcaaaaatgaagtaggagtactcaggaaaacgcgacatgtgaatatcctcctcttcatgggttattcaacaaagccacaactggctattgttacccagtggtgtgagggctccagtttatatcatcatctccacatcattgagaccaaattcgagatgatcaaacttatagatattgcacggcagactgcacagggcatggattacttacacgccaagtcaatcatccacagagacctcaagagtaataatatttttcttcatgaagacctcacagtaaaaataggtgattttggtctagccacagtgaaatctcgatggagtgggtcccatcagtttgaacagttgtctggatccattttgtggatggcaccagaagtaatcagaatgcaagataaaaacccatatagctttcagtcagatgtatatgcatttgggattgttctgtatgaattgatgaccggacagttaccttattcaaatatcaacaacagggaccagataatttttatggtgggacgaggatatctgtctccagatctcagtaaggtacggagtaactgtccaaaagccatgaagagattaatggcagagtgcctaaaaaagaaaagagatgaaagaccactctttccccaaattctcgcctctattgagctgctggcccgctcattgccaaaaattcaccgcagtgcatcagaaccctccttgaatcgggctggcttccaaacagaggattttagtctatatgcttgtgcttctccaaaaacacccattcaggcagggggatatggagaatttgcagccttcaagtagccacaccatcatgacagcatctactcttatttcttaagtcttgtgttcgtacaatttgttaacatcaaaacacagttctgttcctcaactctttttaaagttaaaatttttcagtgcataagctggtgtggaacagaaggaaatttcccatccaacaaaagagggaagaatgttttaggaaccagaattctctgctgccagtgtttcttcttcaacacaaatatcacaagtctgcccactcccaggaagaaagaggagagaccctgagttctgaccttttgatggtcaggcatgatggaaagaaactgctgctacagcttgggagatttgctctgggaagtctgccagtcaactttgcccttctaaccaccagatcaatatgtggctgatcatctgatggggcagttgcaatcaccaagccttgttctctttcctgttctgggattgtgttgtggaacccttttccctagccaccaccagttcatttctgagggatggaacaaaaatgcagcatgcccttcctgtgtggtgcatgttcagtccttgacaaatttttaccaaaatgaagctactttatttaaaaggagggtgagaggtgaggaggtcactttgggtgtggcggaaagggaatgctgcatctttttcctgggctgctggggctctggccttggcttgccagccggaagcgctggcacgcatcgccttcttttcccattgggtccagcaatgaagacgagtgtttggggttttttttttctccaccatgtagcaagttctcaggaaaatacaattgatatcttcctcctaagctcttccaatcagtcaccaagtacttatgtggttactttgtccagggcacaaaatgcctgtatctaattaaaagcctacaaaactgcttgataacagttttgaatgtgagacatttatgtaatttaaatgtaaggtacaagttttaatttctgagtttcttctattatatttttattaaaaaaagaaaataattttcagattgaattggagtaaaataatattacttcccactagaattatatatcctggaaaattgtatttttgttacataagcagcttttaaagaaagatcattacccttttctctacataaatatatggggagtcttagcctaatgacaaatatttataatttttaaattaatggtacttgctggatccatactaacatctttactaatacctcattgtttcttccaacttactcctacactacatcctacatcttcttcctagtcttttatctagaatatgcaacctcaaataaaaatggtggtgtcctcattcattctcctccttccttttttcccaagcctgatcttcaaaaggttggttaatttggcagctgagttcctccccaggcagagaatagaccaattttaggtgtattgggactgagggaggatgtgtaaagattaacatcagtaaagaaccgctgtggagtaattaagaactttgttctttataactggagaatataacctaaccctaacatccctcagcctttactaaagtgtggcgtaaatcacagtagtagcaaagaaagtgactctggatgtgttcctggccagtacctcccttatcatgaatgtagactctctcatcaagatttaggaatataaatcaaatcaaatgtgcccagccaagctatgtagtaagggacttgaacaatattaggcagaacctataaaataaatcagggaattagaaattatttaaagttttcaaattgtaaattgccccggtgtctttcagcctactgccattatttttgctacaatacctacatttcagaggagggcctactgaaaattccatgcaagtggaaaataatcctcaagttattaatgagtttgaaaagcaatgagttcttaagtctttgtgagtagagcaagatcctacaaaattcagaaatagtaaaaatggattcatgctgatttgaagagcatctgtgtgcataatataatgctgcatctcttttaaaagcagtctatttttctttttaaatttgtccccatagatgcttttgaacatgaacatgcttatgttaccttttccgaggttgggaagagccaggagctctcaggcagggccccctccctcagctgggcaggagctgctcaggaggagctagttatagaggaagcttagcgttggcattttcaaaattcaaggtgataacgctttcttcttcctttctgttttagaatagattgctgtctgatttgaaaaagggaaatagatttgatctcaaatgaatctgtgcccagaagccaggctcagggtattcagagatttgtatagtgccctcaaaaaataacaaaattttagctttccttttttcttcttttctccatcaaattcttttttctctagtttacaaatgacatggaaaaggaatttcccctgagttttgtatgcctttttttttttggcttagactatagataggcgtgttgagctcctaagaaaatacaaggaggaactctttgttgtgcagagcactttatgagtagtttgtgtggataatatgtgactgcttccctgacgagcttgtgaggctgtacttatgtctttcctgtaaggcagcttcagtgccttctgtagtgtatataaggaaagattacgccttctgaaaaatctcagagcaaccataagattattttaaaatatgtagtatgactgatggactttttcatcattaaattagtctagcatctaaacttttaccactgaaataatattgaccaaaaagcaatttataaaaggtatttgtgaatagaaaatacaatgtgatcatttgtacttatgtgcaccttaaaagaggaattctgtctagctgtcaaattctggttccttaacatccagtccttgattgtgattgagatctggtaggacgtgctggggcacgctagcagataaaatcccgtatactttaggatagatgttacatttatgtcagtgttggcaaagagcattgtgtagtaataaagaattcaagacttcagcaatgtcaacctgaaactttgtaaatatttcctagattgttatttgatgcagtcacagctctttatcacacaatgttgtctttccctcatcaggcaattttagaactgctgcacacccctcctcagatctcacctgcccctcctgtacattcacctctccagccttgtgcacacctcatttagctttagtttgaaacacattgcagggttcaggtgacctcttcaaaaactacctcctcagaatgaggtaatgaatagttatttattttaaaatatgaaaagtcaggagctctagaatatgaagatgatctaagattttaacttttatgtatacttgttgagcactctccttttgtcctaaagggcattatacatttaagcagtaatactgaaaaatgtagctcagagtaactgaatgttgttgaaagtggtgccagaatctgttttaggggtacgtatcagaatcttaatcttaaatcggttacatgaaattaaatagttaatggtaacacttgactaacagatataattttaattttcggtaggcttttagcaagacagtaagtacatcttcataatgagttagccacagcttcatcacatgcacagattttcctgttgagagactgcccagttaagagggtagaatgatgaaccatttttcaggattctcttctttgtccaaactggcattgtgagtgctagaatatcagcactttcaaactagtgattccaactattaggctattaaaaagcaaaacaaaccaaacaaaccatagccagacatgggaagtttactatgagtataaacagcaaatagcttacaggtcatacattgaaatggtgtaggtaaggcgttagaaaaataccttgacaatttgccaaatgatcttactgtgccttcatgatgcaataaaaaaaaaaaaaatttagcataaatcagtgatttgtgaagagagcagccaccctggtctaactcagctgtgttaatattttttagcgtgcaatttagactgcaaagataaatgcactaaagagtttatagccaaaatcacatttaaaaaatgagagaaaacacaggtaaattttcagtgaacaaaattatttttttaaagtacataatccctagtatagtcagatatatttatcacatagagcaaataggttgaaatcacaattcagtgacatttctagagaaactttttctactcccataggttcttcaaagcatggaacttttatataacagaaatgtgtgacggtcattttaaattgctgtagtttggggctgaagtactgtgtgctgggcagcaatcacatgtattaactagtgagaaaggagaaattaagatataggacagaatttgattttcttgttcccagattactgctgccaacctagacactgagtttccagaggctgaaacgtaaacttgcagctcagcaactgttttgcaaagttagtgggactgtcctgcttatgctgttcaaaaatgctctgagggccaggtggggcctccaggggctcctctctgaggggacatcagactagctaacgacctggcgggcggatgtgaaccggacacactccatggtgtgcttcttgtatcggtccctcgccaccctcaagaaaggcttcagcgggttctctagacgtctccactaaggtgtgttactaacagccatgggttgttgagcacccgaggagtgcaatagcatctctgcatgattgtatattggcccgaagagaatgaagtggccagtgtactcatgttccatgttgctagctctggtaaactgaaaatactggtaagatttttgttttatcagtacactagagagtaagctttgttttgttgtttttagataatgttttcacttccatttggaaagacatttaaattgagtttcagtcctaaattttgccagtcatggtaattagcagtttctatcaggtatttttaaggtagaagaggatagaaacataagttctaaaagcttaaggtaaccgtggtttattttaaaatgtttaggggtggttagtctctacctcaaaaaaagtgagtgaatcttttatttcagcattcacaagttcggctgttgtttttgtaatacattttttttttaaccttttgacccccctttacctaagtgtcaatgtagttttattaattactaagtcagtttcattaaaatgtttatttagcagttttgactaattgcaatgattaatatagccagttgtgcatgaggacacagccagtgagtatatctgggttttttttgtgatgctttttttcttaagacttctgtagatttatgaagtactcattgaaaacaactaaaatacgtttattcgtgttaatatggaaaaaaaaaaa

SEQ ID NO: 24 - protein, 766 aa, Bos taurus
MAALSGGGGGGGGGAEQGQALFNGDMEPEAGAAASSAADPAIPEEVWNIKQMIKLTQEHIEALLDKFGGEHNPPSIYLEAYEEYTSKLDALQQREQQLLESLGNGTDFSVSSSASTDTVTSSSSSSLSVLPSSLSVFQNPTDVSRSNPKSPQKPIVRVFLPNKQRTVVPARCGVTVRDSLKKALMMRGLIPECCAVYRIQDGEKKPIGWDTDISWLTGEELHVEVLENVPLTTHNFVRKTFFTLAFCDFCRKLLFQGFRCQTCGYKFHQRCSTEVPLMCVNYDQLDLLFVSKFFEHHPIPQEEASLAETTLPCGSSPSAPPSDSIGPPILTSPSPSKSIPIPQPFRPADEDHRNQFGQRDRSSSAPNVHINTIEPVNIDDLIRDQGFRSDGGSTTGLSATPPASLPGSLSNVKALQKSPGPQRERKSSSSSEDRNRMKTLGRRDSSDDWEIPDGQITVGQRIGSGSFGTVYKGKWHGDVAVKMLNVTAPTPQQLQAFKNEVGVLRKTRHVNILLFMGYSTKPQLAIVTQWCEGSSLYHHLHIIETKFEMIKLIDIARQTAQGMDYLHAKSIIHRDLKSNNIFLHEDLTVKIGDFGLATVKSRWSGSHQFEQLSGSILWMAPEVIRMQDKNPYSFQSDVYAFGIVLYELMTGQLPYSNINNRDQIIFMVGRGYLSPDLSKVRSNCPKAMKRLMAECLKKKRDERPLFPQILASIELLARSLPKIHRSASEPSLNRAGFQTEDFSLYACASPKTPIQAGGYGEFAAFK

SEQ ID NO: 25 - DNA, 4670 bp, Bos taurus
ggtgtgtcatagtgcagcagattgaatgcagaagatatgaaaattcagatgtcttctgttaaggtgtggaatatcaaacaaatgattaagttgacacaggagcatatagaggccctattggacaaatttggtggggagcataatccaccatcaatatatctggaggcctatgaagaatacaccagcaagctagatgccctccaacaaagagaacaacagttattggaatccctggggaatggaactgatttttctgtttctagctctgcatcaacggacaccgttacatcttcttcctcttctagcctttcagtgctgccttcatctctttcagtttttcaaaatcccacagatgtgtcacggagcaaccccaagtcaccacaaaaacctatcgttagagtcttcctgcccaataaacagaggacagtggtacctgcacggtgtggagtcacagtccgggacagcctgaagaaggcactgatgatgagaggtctaatcccagagtgctgtgctgtttacagaattcaggatggggagaagaaaccaattggctgggacactgatatttcctggcttactggagaggagttgcatgtagaagtgttggagaatgttccacttacaacacacaactttgtacggaaaacttttttcaccttagcattttgtgacttctgtagaaagctgcttttccagggattccgctgtcaaacatgtggttataaatttcaccagcgttgtagtacagaggttccactgatgtgtgttaattatgaccaactagatttgctgtttgtctccaagttctttgaacaccacccaataccacaggaggaggcctccttagcagagactacccttccatgtggctcatccccttctgcacccccctccgattctattgggcccccaattctcaccagtccatctccttcaaaatccattccaattccacagcctttccgaccagcagatgaagatcatcgaaatcagtttggacaacgagaccggtcctcatcagctccaaatgtgcatataaacacaatagaacccgtcaatattgatgacttgattagagaccaagggtttcgtagtgatggaggatcaaccacaggtttatccgccacaccccctgcctcattacctggctcactctctaatgtgaaagcattgcagaaatctccaggacctcagcgagaaagaaagtcctcttcatcctcagaagacaggaatcgaatgaaaacgcttggtagacgggattcaagtgacgattgggagattcctgatggacagatcacagtgggacaaagaattggatcagggtcatttgggacagtctacaagggaaagtggcatggtgatgtggcagtgaaaatgttgaatgtgacagcacccacacctcagcagttacaggccttcaaaaatgaagtaggagtactcaggaaaacgcgacatgtgaatatcctcctcttcatgggttattcaacaaagccacaactggctattgttacccagtggtgtgagggctccagtttatatcatcatctccacatcattgagaccaaattcgagatgatcaaacttatagatattgcacggcagactgcacagggcatggattacttacacgccaagtcaatcatccacagagacctcaagagtaataatatttttcttcatgaagacctcacagtaaaaataggtgattttggtctagccacagtgaaatctcgatggagtgggtcccatcagtttgaacagttgtctggatccattttgtggatggcaccagaagtaatcagaatgcaagataaaaacccatatagctttcagtcagatgtatatgcatttgggattgttctgtatgaattgatgaccggacagttaccttattcaaatatcaacaacagggaccagataatttttatggtgggacgaggatatctgtctccagatctcagtaaggtacggagtaactgtccaaaagccatgaagagattaatggcagagtgcctaaaaaagaaaagagatgaaagaccactctttccccaagtaggaaagactctcctaagcaagagacaaaattcagaagttatcagggaaaaagataagcagattctcgcctctattgagctgctggcccgctcattgccaaaaattcaccgcagtgcatcagaaccctccttgaatcgggctggcttccaaacagaggattttagtctatatgcttgtgcttctccaaaaacacccattcaggcagggggatatgaagcagatttggctcttacatcaaataaaaatagagtagaagttgggatttagagatttcctgacatgcaagaaggaataagcaagaaaaaaaggtttgttttccccaaatcatatctattgtcttttacttctattttttcttaaattttttgtgatttcagagacatgtagagttttattgatacctaaactatgagttcttttttttttttttttttcattattttgatttttttggccaagaggcatatgggatcttagcttgagaaagcaacaattttcttgatgtcattttgggtgagggcacatattgctgtgaacagtgtggtgatagccaccagggaccaaactcacacccgctgcattgaaaggtgaagtcttaaacactggaccagcagagaaattcctactctatgagttctttttgtcatcccctccccgcaccctccacccccaacctaaagtctgatgatgaaatcaacaactattccattagaagcagtagattctggtagcatgatctttagtttgttagtaagattttgtgctttgtggggttgtgtcgttttaaggctaatatttaagtttgtcaaatagaatgctgttcagattgtaaaaatgagtaataaacatctgaagttttttttaagttatttttaacatggtatatacagttgagcttagagtttatcattttctgatattctcttacttagtagatgaattctagccattttttataaagatttctgttaagcaaatcctgttttcacatgggcttcctttaagggattttagattctgctggatatggtgactgctcataagactgttgaaaattacttttaagatgtattagaatacttctgaaaaaaaatagcaaccttaaaaccataagcaaaagtagtaagggtgtttatacatttctagagtccctgtttaggtaatagcctcctatgattgtactttaaatgttttgctctccaaggttttagtaacttggctttttttctaatcagtgccaaactcccccagtttttttaactttaaatatgaggtaataaatcttttacccttccttgatcttttgacttataataccttggtcagttgtttcttaaaaggaatccttaaatggaaagagacaatatcactgtctgcagttctgattagtagttttattcagaatggaaaaacagattattcatttttgaaaattgttcaggggtatgttcattgttaggaccttggactttggagtcagtgcctagctatgcattccaggtctgccattttctggctgtgaaattttggacaagttacttaaccactttaaaccccagctttaagaagtaaattaaccccagtaaattaagaagtaatagcagccacttcgtagagttgttatgaggctcagatgcagtgcaaatgtgtataaagtattcagggagtcacctggtatactataatagacactagaatagttgccaatattatcagcatacaatctgaggattctgtcagccaatcattagcaatctgttgtttgttgggacatgccagtgttctccagttgaaatcagtagcaatctaaaaatggatagattattcctcatttaaatagtgtgttcatataagtgattgcttggatccttatcagaagttgctgttactgaaaaatgataaggctgactaaattgtgatagttgtcagttactaaccaactcccagaaatgaataagaggaacctatctctagttcctagtagaaggtatggacaaaatagtaggtgaaaaataatgtcttgaacccccaaattaagtaagctttaaagagtacaatacctcaaagggtctttgcggtttaaaatttgtatgctgagaatgatgttcattgacatgtgcctatatgtaattttttgatagtttaaaaggtgaaatgaactacagatgggagaggtctgaattttcttgccttcagtcaaatgtgtaatgtggacatattatttgacctgtgaattttatcttttaaaaaagattaattcctgcttcttccttcctaatagttgcattataataatgaaaatgagttgataatttggggggaaagtattctacaaatcaaccttattattttaccattggtttctgagaaattttgttcatttgaaccgtttatagcttgattagaatcatagcatgtaaaacccaactgagggattatctgcagacttaatgtagtattatgtaagttgtcttctttcatttcgaccttttttgcttttgttgttgctagatctgtagtatgtagctagtcacctttcagcgaggtttcagcgaggcttttctgtgtctctaggttatttgagataacttttttaaaattagctcttgtcctcc

SEQ ID NO: 26 - protein, 761 aa, Bos taurus
MKIQMSSVKVWNIKQMIKLTQEHIEALLDKFGGEHNPPSIYLEAYEEYTSKLDALQQREQQLLESLGNGTDFSVSSSASTDTVTSSSSSSLSVLPSSLSVFQNPTDVSRSNPKSPQKPIVRVFLPNKQRTVVPARCGVTVRDSLKKALMMRGLIPECCAVYRIQDGEKKPIGWDTDISWLTGEELHVEVLENVPLTTHNFVRKTFFTLAFCDFCRKLLFQGFRCQTCGYKFHQRCSTEVPLMCVNYDQLDLLFVSKFFEHHPIPQEEASLAETTLPCGSSPSAPPSDSIGPPILTSPSPSKSIPIPQPFRPADEDHRNQFGQRDRSSSAPNVHINTIEPVNIDDLIRDQGFRSDGGSTTGLSATPPASLPGSLSNVKALQKSPGPQRERKSSSSSEDRNRMKTLGRRDSSDDWEIPDGQITVGQRIGSGSFGTVYKGKWHGDVAVKMLNVTAPTPQQLQAFKNEVGVLRKTRHVNILLFMGYSTKPQLAIVTQWCEGSSLYHHLHIIETKFEMIKLIDIARQTAQGMDYLHAKSIIHRDLKSNNIFLHEDLTVKIGDFGLATVKSRWSGSHQFEQLSGSILWMAPEVIRMQDKNPYSFQSDVYAFGIVLYELMTGQLPYSNINNRDQIIFMVGRGYLSPDLSKVRSNCPKAMKRLMAECLKKKRDERPLFPQVGKTLLSKRQNSEVIREKDKQILASIELLARSLPKIHRSASEPSLNRAGFQTEDFSLYACASPKTPIQAGGYEADLALTSNKNRVEVGI

SEQ ID NO: 27 - DNA, 4816 bp, Bos taurus
ctcagctgcgccgggtctcacaagacggttcccgaggtggcccaggcgccgtcccaccgccgacgccgcccgggccgcccgggccgtccctccccgctgccccccgtcctccgcctccgcctccccccgccctcagcctcccttccccctccccgcccagcagcggtcgctcgggcccggctctcggttataagatggcggcgctgagtggcggcggcggcggcggcggcggtggcgcggagcagggccaggctctgttcaacggggacatggagcccgaggccggcgccgcggcctcttcggctgcggaccccgccattcccgaggaggtgtggaatatcaaacaaatgattaagttgacacaggagcatatagaggccctattggacaaatttggtggggagcataatccaccatcaatatatctggaggcctatgaagaatacaccagcaagctagatgccctccaacaaagagaacaacagttattggaatccctggggaatggaactgatttttctgtttctagctctgcatcaacggacaccgttacatcttcttcctcttctagcctttcagtgctgccttcatctctttcagtttttcaaaatcccacagatgtgtcacggagcaaccccaagtcaccacaaaaacctatcgttagagtcttcctgcccaataaacagaggacagtggtacctgcacggtgtggagtcacagtccgggacagcctgaagaaggcactgatgatgagaggtctaatcccagagtgctgtgctgtttacagaattcaggatggggagaagaaaccaattggctgggacactgatatttcctggcttactggagaggagttgcatgtagaagtgttggagaatgttccacttacaacacacaactttgtacggaaaacttttttcaccttagcattttgtgacttctgtagaaagctgcttttccagggattccgctgtcaaacatgtggttataaatttcaccagcgttgtagtacagaggttccactgatgtgtgttaattatgaccaactagagcccccaattctcaccagtccatctccttcaaaatccattccaattccacagcctttccgaccagcagatgaagatcatcgaaatcagtttggacaacgagaccggtcctcatcagctccaaatgtgcatataaacacaatagaacccgtcaatattgatgacttgattagagaccaagggtttcgtagtgatggaggatcaaccacaggtttatccgccacaccccctgcctcattacctggctcactctctaatgtgaaagcattgcagaaatctccaggacctcagcgagaaagaaagtcctcttcatcctcagaagacaggaatcgaatgaaaacgcttggtagacgggattcaagtgacgattgggagattcctgatggacagatcacagtgggacaaagaattggatcagggtcatttgggacagtctacaagggaaagtggcatggtgatgtggcagtgaaaatgttgaatgtgacagcacccacacctcagcagttacaggccttcaaaaatgaagtaggagtactcaggaaaacgcgacatgtgaatatcctcctcttcatgggttattcaacaaagccacaactggctattgttacccagtggtgtgagggctccagtttatatcatcatctccacatcattgagaccaaattcgagatgatcaaacttatagatattgcacggcagactgcacagggcatggattacttacacgccaagtcaatcatccacagagacctcaagagtaataatatttttcttcatgaagacctcacagtaaaaataggtgattttggtctagccacagtgaaatctcgatggagtgggtcccatcagtttgaacagttgtctggatccattttgtggatggcaccagaagtaatcagaatgcaagataaaaacccatatagctttcagtcagatgtatatgcatttgggattgttctgtatgaattgatgaccggacagttaccttattcaaatatcaacaacagggaccagataatttttatggtgggacgaggatatctgtctccagatctcagtaaggtacggagtaactgtccaaaagccatgaagagattaatggcagagtgcctaaaaaagaaaagagatgaaagaccactctttccccaagtaggaaagactctcctaagcaagagacaaaattcagaagttatcagggaaaaagataagcagattctcgcctctattgagctgctggcccgctcattgccaaaaattcaccgcagtgcatcagaaccctccttgaatcgggctggcttccaaacagaggattttagtctatatgcttgtgcttctccaaaaacacccattcaggcagggggatatgaagcagatttggctcttacatcaaataaaaatagagtagaagttgggatttagagatttcctgacatgcaagaaggaataagcaagaaaaaaaggtttgttttccccaaatcatatctattgtcttttacttctattttttcttaaattttttgtgatttcagagacatgtagagttttattgatacctaaactatgagttcttttttttttttttttttcattattttgatttttttggccaagaggcatatgggatcttagcttgagaaagcaacaattttcttgatgtcattttgggtgagggcacatattgctgtgaacagtgtggtgatagccaccagggaccaaactcacacccgctgcattgaaaggtgaagtcttaaacactggaccagcagagaaattcctactctatgagttctttttgtcatcccctccccgcaccctccacccccaacctaaagtctgatgatgaaatcaacaactattccattagaagcagtagattctggtagcatgatctttagtttgttagtaagattttgtgctttgtggggttgtgtcgttttaaggctaatatttaagtttgtcaaatagaatgctgttcagattgtaaaaatgagtaataaacatctgaagttttttttaagttatttttaacatggtatatacagttgagcttagagtttatcattttctgatattctcttacttagtagatgaattctagccattttttataaagatttctgttaagcaaatcctgttttcacatgggcttcctttaagggattttagattctgctggatatggtgactgctcataagactgttgaaaattacttttaagatgtattagaatacttctgaaaaaaaatagcaaccttaaaaccataagcaaaagtagtaagggtgtttatacatttctagagtccctgtttaggtaatagcctcctatgattgtactttaaatgttttgctctccaaggttttagtaacttggctttttttctaatcagtgccaaactcccccagtttttttaactttaaatatgaggtaataaatcttttacccttccttgatcttttgacttataataccttggtcagttgtttcttaaaaggaatccttaaatggaaagagacaatatcactgtctgcagttctgattagtagttttattcagaatggaaaaacagattattcatttttgaaaattgttcaggggtatgttcattgttaggaccttggactttggagtcagtgcctagctatgcattccaggtctgccattttctggctgtgaaattttggacaagttacttaaccactttaaaccccagctttaagaagtaaattaaccccagtaaattaagaagtaatagcagccacttcgtagagttgttatgaggctcagatgcagtgcaaatgtgtataaagtattcagggagtcacctggtatactataatagacactagaatagttgccaatattatcagcatacaatctgaggattctgtcagccaatcattagcaatctgttgtttgttgggacatgccagtgttctccagttgaaatcagtagcaatctaaaaatggatagattattcctcatttaaatagtgtgttcatataagtgattgcttggatccttatcagaagttgctgttactgaaaaatgataaggctgactaaattgtgatagttgtcagttactaaccaactcccagaaatgaataagaggaacctatctctagttcctagtagaaggtatggacaaaatagtaggtgaaaaataatgtcttgaacccccaaattaagtaagctttaaagagtacaatacctcaaagggtctttgcggtttaaaatttgtatgctgagaatgatgttcattgacatgtgcctatatgtaattttttgatagtttaaaaggtgaaatgaactacagatgggagaggtctgaattttcttgccttcagtcaaatgtgtaatgtggacatattatttgacctgtgaattttatcttttaaaaaagattaattcctgcttcttccttcctaatagttgcattataataatgaaaatgagttgataatttggggggaaagtattctacaaatcaaccttattattttaccattggtttctgagaaattttgttcatttgaaccgtttatagcttgattagaatcatagcatgtaaaacccaactgagggattatctgcagacttaatgtagtattatgtaagttgtcttctttcatttcgaccttttttgcttttgttgttgctagatctgtagtatgtagctagtcacctttcagcgaggtttcagcgaggcttttctgtgtctctaggttatttgagataacttttttaaaattagctcttgtcctcc

SEQ ID NO: 28 - protein, 757 aa, Bos taurus
MAALSGGGGGGGGGAEQGQALFNGDMEPEAGAAASSAADPAIPEEVWNIKQMIKLTQEHIEALLDKFGGEHNPPSIYLEAYEEYTSKLDALQQREQQLLESLGNGTDFSVSSSASTDTVTSSSSSSLSVLPSSLSVFQNPTDVSRSNPKSPQKPIVRVFLPNKQRTVVPARCGVTVRDSLKKALMMRGLIPECCAVYRIQDGEKKPIGWDTDISWLTGEELHVEVLENVPLTTHNFVRKTFFTLAFCDFCRKLLFQGFRCQTCGYKFHQRCSTEVPLMCVNYDQLEPPILTSPSPSKSIPIPQPFRPADEDHRNQFGQRDRSSSAPNVHINTIEPVNIDDLIRDQGFRSDGGSTTGLSATPPASLPGSLSNVKALQKSPGPQRERKSSSSSEDRNRMKTLGRRDSSDDWEIPDGQITVGQRIGSGSFGTVYKGKWHGDVAVKMLNVTAPTPQQLQAFKNEVGVLRKTRHVNILLFMGYSTKPQLAIVTQWCEGSSLYHHLHIIETKFEMIKLIDIARQTAQGMDYLHAKSIIHRDLKSNNIFLHEDLTVKIGDFGLATVKSRWSGSHQFEQLSGSILWMAPEVIRMQDKNPYSFQSDVYAFGIVLYELMTGQLPYSNINNRDQIIFMVGRGYLSPDLSKVRSNCPKAMKRLMAECLKKKRDERPLFPQVGKTLLSKRQNSEVIREKDKQILASIELLARSLPKIHRSASEPSLNRAGFQTEDFSLYACASPKTPIQAGGYEADLALTSNKNRVEVGI

SEQ ID NO: 29 - DNA, 2499 bp, Bos taurus
ctcagctgcgccgggtctcacaagacggttcccgaggtggcccaggcgccgtcccaccgccgacgccgcccgggccgcccgggccgtccctccccgctgccccccgtcctccgcctccgcctccccccgccctcagcctcccttccccctccccgcccagcagcggtcgctcgggcccggctctcggttataagatggcggcgctgagtggcggcggcggcggcggcggcggtggcgcggagcagggccaggctctgttcaacggggacatggagcccgaggccggcgccgcggcctcttcggctgcggaccccgccattcccgaggaggtgtggaatatcaaacaaatgattaagttgacacaggagcatatagaggccctattggacaaatttggtggggagcataatccaccatcaatatatctggaggcctatgaagaatacaccagcaagctagatgccctccaacaaagagaacaacagttattggaatccctggggaatggaactgatttttctgtttctagctctgcatcaacggacaccgttacatcttcttcctcttctagcctttcagtgctgccttcatctctttcagtttttcaaaatcccacagatgtgtcacggagcaaccccaagtcaccacaaaaacctatcgttagagtcttcctgcccaataaacagaggacagtggtacctgcacggtgtggagtcacagtccgggacagcctgaagaaggcactgatgatgagaggtctaatcccagagtgctgtgctgtttacagaattcaggatggggagaagaaaccaattggctgggacactgatatttcctggcttactggagaggagttgcatgtagaagtgttggagaatgttccacttacaacacacaactttgtacggaaaacttttttcaccttagcattttgtgacttctgtagaaagctgcttttccagggattccgctgtcaaacatgtggttataaatttcaccagcgttgtagtacagaggttccactgatgtgtgttaattatgaccaactagatttgctgtttgtctccaagttctttgaacaccacccaataccacaggaggaggcctccttagcagagactacccttccatgtggctcatccccttctgcacccccctccgattctattgggcccccaattctcaccagtccatctccttcaaaatccattccaattccacagcctttccgaccagcagatgaagatcatcgaaatcagtttggacaacgagaccggtcctcatcagctccaaatgtgcatataaacacaatagaacccgtcaatattgatgacttgattagagaccaagggtttcgtagtgatggaggatcaaccacaggtttatccgccacaccccctgcctcattacctggctcactctctaatgtgaaagcattgcagaaatctccaggacctcagcgagaaagaaagtcctcttcatcctcagaagacaggaatcgaatgaaaacgcttggtagacgggattcaagtgacgattgggagattcctgatggacagatcacagtgggacaaagaattggatcagggtcatttgggacagtctacaagggaaagtggcatggtgatgtggcagtgaaaatgttgaatgtgacagcacccacacctcagcagttacaggccttcaaaaatgaagtaggagtactcaggaaaacgcgacatgtgaatatcctcctcttcatgggttattcaacaaagccacaactggctattgttacccagtggtgtgagggctccagtttatatcatcatctccacatcattgagaccaaattcgagatgatcaaacttatagatattgcacggcagactgcacagggcatggattacttacacgccaagtcaatcatccacagagacctcaagagtaataatatttttcttcatgaagacctcacagtaaaaataggtgattttggtctagccacagtgaaatctcgatggagtgggtcccatcagtttgaacagttgtctggatccattttgtggatggcaccagaagtaatcagaatgcaagataaaaacccatatagctttcagtcagatgtatatgcatttgggattgttctgtatgaattgatgaccggacagttaccttattcaaatatcaacaacagggaccagataatttttatggtgggacgaggatatctgtctccagatctcagtaaggtacggagtaactgtccaaaagccatgaagagattaatggcagagtgcctaaaaaagaaaagagatgaaagaccactctttccccaagtaggaaagactctcctaagcaagagacaaaattcagaagttatcagggaaaaagataagcaggaaaagtatgtttctttagtacattccaggcatttgggattacagtaaaaacaatattctcgcctctattgagctgctggcccgctcattgccaaaaattcaccgcagtgcatcagaa

SEQ ID NO: 30 - protein, 744 aa, Bos taurus
MAALSGGGGGGGGGAEQGQALFNGDMEPEAGAAASSAADPAIPEEVWNIKQMIKLTQEHIEALLDKFGGEHNPPSIYLEAYEEYTSKLDALQQREQQLLESLGNGTDFSVSSSASTDTVTSSSSSSLSVLPSSLSVFQNPTDVSRSNPKSPQKPIVRVFLPNKQRTVVPARCGVTVRDSLKKALMMRGLIPECCAVYRIQDGEKKPIGWDTDISWLTGEELHVEVLENVPLTTHNFVRKTFFTLAFCDFCRKLLFQGFRCQTCGYKFHQRCSTEVPLMCVNYDQLDLLFVSKFFEHHPIPQEEASLAETTLPCGSSPSAPPSDSIGPPILTSPSPSKSIPIPQPFRPADEDHRNQFGQRDRSSSAPNVHINTIEPVNIDDLIRDQGFRSDGGSTTGLSATPPASLPGSLSNVKALQKSPGPQRERKSSSSSEDRNRMKTLGRRDSSDDWEIPDGQITVGQRIGSGSFGTVYKGKWHGDVAVKMLNVTAPTPQQLQAFKNEVGVLRKTRHVNILLFMGYSTKPQLAIVTQWCEGSSLYHHLHIIETKFEMIKLIDIARQTAQGMDYLHAKSIIHRDLKSNNIFLHEDLTVKIGDFGLATVKSRWSGSHQFEQLSGSILWMAPEVIRMQDKNPYSFQSDVYAFGIVLYELMTGQLPYSNINNRDQIIFMVGRGYLSPDLSKVRSNCPKAMKRLMAECLKKKRDERPLFPQVGKTLLSKRQNSEVIREKDKQEKYVSLVHSRHLGLQ

SEQ ID NO: 31 - DNA, 2404 bp, Bos taurus
ctcagctgcgccgggtctcacaagacggttcccgaggtggcccaggcgccgtcccaccgccgacgccgcccgggccgcccgggccgtccctccccgctgccccccgtcctccgcctccgcctccccccgccctcagcctcccttccccctccccgcccagcagcggtcgctcgggcccggctctcggttataagatggcggcgctgagtggcggcggcggcggcggcggcggtggcgcggagcagggccaggctctgttcaacggggacatggagcccgaggccggcgccgcggcctcttcggctgcggaccccgccattcccgaggaggtgtggaatatcaaacaaatgattaagttgacacaggagcatatagaggccctattggacaaatttggtggggagcataatccaccatcaatatatctggaggcctatgaagaatacaccagcaagctagatgccctccaacaaagagaacaacagttattggaatccctggggaatggaactgatttttctgtttctagctctgcatcaacggacaccgttacatcttcttcctcttctagcctttcagtgctgccttcatctctttcagtttttcaaaatcccacagatgtgtcacggagcaaccccaagtcaccacaaaaacctatcgttagagtcttcctgcccaataaacagaggacagtggtacctgcacggtgtggagtcacagtccgggacagcctgaagaaggcactgatgatgagaggtctaatcccagagtgctgtgctgtttacagaattcaggatggggagaagaaaccaattggctgggacactgatatttcctggcttactggagaggagttgcatgtagaagtgttggagaatgttccacttacaacacacaactttgtacggaaaacttttttcaccttagcattttgtgacttctgtagaaagctgcttttccagggattccgctgtcaaacatgtggttataaatttcaccagcgttgtagtacagaggttccactgatgtgtgttaattatgaccaactagatttgctgtttgtctccaagttctttgaacaccacccaataccacaggaggaggcctccttagcagagactacccttccatgtggctcatccccttctgcacccccctccgattctattgggcccccaattctcaccagtccatctccttcaaaatccattccaattccacagcctttccgaccagcagatgaagatcatcgaaatcagtttggacaacgagaccggtcctcatcagctccaaatgtgcatataaacacaatagaacccgtcaatattgatgacttgattagagaccaagggtttcgtagtgatggaggatcaaccacaggtttatccgccacaccccctgcctcattacctggctcactctctaatgtgaaagcattgcagaaatctccaggacctcagcgagaaagaaagtcctcttcatcctcagaagacaggaatcgaatgaaaacgcttggtagacgggattcaagtgacgattgggagattcctgatggacagatcacagtgggacaaagaattggatcagggtcatttgggacagtctacaagggaaagtggcatggtgatgtggcagtgaaaatgttgaatgtgacagcacccacacctcagcagttacaggccttcaaaaatgaagtaggagtactcaggaaaacgcgacatgtgaatatcctcctcttcatgggttattcaacaaagccacaactggctattgttacccagtggtgtgagggctccagtttatatcatcatctccacatcattgagaccaaattcgagatgatcaaacttatagatattgcacggcagactgcacagggcatggattacttacacgccaagtcaatcatccacagagacctcaagagtaataatatttttcttcatgaagacctcacagtaaaaataggtgattttggtctagccacagtgaaatctcgatggagtgggtcccatcagtttgaacagttgtctggatccattttgtggatggcaccagaagtaatcagaatgcaagataaaaacccatatagctttcagtcagatgtatatgcatttgggattgttctgtatgaattgatgaccggacagttaccttattcaaatatcaacaacagggaccagataatttttatggtgggacgaggatatctgtctccagatctcagtaaggtacggagtaactgtccaaaagccatgaagagattaatggcagagtgcctaaaaaagaaaagagatgaaagaccactctttccccaagatctctcttcccaccatagacacaaaaatttcagatggctacaggtttacatgtaaaaaacagaattataacaaatgatttttat

SEQ ID NO: 32 - protein, 726 aa, Bos taurus
MAALSGGGGGGGGGAEQGQALFNGDMEPEAGAAASSAADPAIPEEVWNIKQMIKLTQEHIEALLDKFGGEHNPPSIYLEAYEEYTSKLDALQQREQQLLESLGNGTDFSVSSSASTDTVTSSSSSSLSVLPSSLSVFQNPTDVSRSNPKSPQKPIVRVFLPNKQRTVVPARCGVTVRDSLKKALMMRGLIPECCAVYRIQDGEKKPIGWDTDISWLTGEELHVEVLENVPLTTHNFVRKTFFTLAFCDFCRKLLFQGFRCQTCGYKFHQRCSTEVPLMCVNYDQLDLLFVSKFFEHHPIPQEEASLAETTLPCGSSPSAPPSDSIGPPILTSPSPSKSIPIPQPFRPADEDHRNQFGQRDRSSSAPNVHINTIEPVNIDDLIRDQGFRSDGGSTTGLSATPPASLPGSLSNVKALQKSPGPQRERKSSSSSEDRNRMKTLGRRDSSDDWEIPDGQITVGQRIGSGSFGTVYKGKWHGDVAVKMLNVTAPTPQQLQAFKNEVGVLRKTRHVNILLFMGYSTKPQLAIVTQWCEGSSLYHHLHIIETKFEMIKLIDIARQTAQGMDYLHAKSIIHRDLKSNNIFLHEDLTVKIGDFGLATVKSRWSGSHQFEQLSGSILWMAPEVIRMQDKNPYSFQSDVYAFGIVLYELMTGQLPYSNINNRDQIIFMVGRGYLSPDLSKVRSNCPKAMKRLMAECLKKKRDERPLFPQDLSSHHRHKNFRWLQVYM

SEQ ID NO: 33 - DNA, 2331 bp, Bos taurus
ctcagctgcgccgggtctcacaagacggttcccgaggtggcccaggcgccgtcccaccgccgacgccgcccgggccgcccgggccgtccctccccgctgccccccgtcctccgcctccgcctccccccgccctcagcctcccttccccctccccgcccagcagcggtcgctcgggcccggctctcggttataagatggcggcgctgagtggcggcggcggcggcggcggcggtggcgcggagcagggccaggctctgttcaacggggacatggagcccgaggccggcgccgcggcctcttcggctgcggaccccgccattcccgaggaggtgtggaatatcaaacaaatgattaagttgacacaggagcatatagaggccctattggacaaatttggtggggagcataatccaccatcaatatatctggaggcctatgaagaatacaccagcaagctagatgccctccaacaaagagaacaacagttattggaatccctggggaatggaactgatttttctgtttctagctctgcatcaacggacaccgttacatcttcttcctcttctagcctttcagtgctgccttcatctctttcagtttttcaaaatcccacagatgtgtcacggagcaaccccaagtcaccacaaaaacctatcgttagagtcttcctgcccaataaacagaggacagtggtacctgcacggtgtggagtcacagtccgggacagcctgaagaaggcactgatgatgagaggtctaatcccagagtgctgtgctgtttacagaattcaggatggggagaagaaaccaattggctgggacactgatatttcctggcttactggagaggagttgcatgtagaagtgttggagaatgttccacttacaacacacaactttgtacggaaaacttttttcaccttagcattttgtgacttctgtagaaagctgcttttccagggattccgctgtcaaacatgtggttataaatttcaccagcgttgtagtacagaggttccactgatgtgtgttaattatgaccaactagatttgctgtttgtctccaagttctttgaacaccacccaataccacaggaggaggcctccttagcagagactacccttccatgtggctcatccccttctgcacccccctccgattctattgggcccccaattctcaccagtccatctccttcaaaatccattccaattccacagcctttccgaccagcagatgaagatcatcgaaatcagtttggacaacgagaccggtcctcatcagctccaaatgtgcatataaacacaatagaacccgtcaatattgatgacttgattagagaccaagggtttcgtagtgatggaggatcaaccacaggtttatccgccacaccccctgcctcattacctggctcactctctaatgtgaaagcattgcagaaatctccaggacctcagcgagaaagaaagtcctcttcatcctcagaagacaggaatcgaatgaaaacgcttggtagacgggattcaagtgacgattgggagattcctgatggacagatcacagtgggacaaagaattggatcagggtcatttgggacagtctacaagggaaagtggcatggtgatgtggcagtgaaaatgttgaatgtgacagcacccacacctcagcagttacaggccttcaaaaatgaagtaggagtactcaggaaaacgcgacatgtgaatatcctcctcttcatgggttattcaacaaagccacaactggctattgttacccagtggtgtgagggctccagtttatatcatcatctccacatcattgagaccaaattcgagatgatcaaacttatagatattgcacggcagactgcacagggcatggattacttacacgccaagtcaatcatccacagagacctcaagagtaataatatttttcttcatgaagacctcacagtaaaaataggtgattttggtctagccacagtgaaatctcgatggagtgggtcccatcagtttgaacagttgtctggatccattttgtggatggcaccagaagtaatcagaatgcaagataaaaacccatatagctttcagtcagatgtatatgcatttgggattgttctgtatgaattgatgaccggacagttaccttattcaaatatcaacaacagggaccaggtgctttgtcctccatgggagtgtaataaatgctgtgcaagggcttacttcccatgagagaagtgagtgaccaacagaaggataatttttatggtgggacgaggatatctgtctccagatctcagtaaggtacggagtaactgtccaa

SEQ ID NO: 34 - protein, 681 aa, Bos taurus
MAALSGGGGGGGGGAEQGQALFNGDMEPEAGAAASSAADPAIPEEVWNIKQMIKLTQEHIEALLDKFGGEHNPPSIYLEAYEEYTSKLDALQQREQQLLESLGNGTDFSVSSSASTDTVTSSSSSSLSVLPSSLSVFQNPTDVSRSNPKSPQKPIVRVFLPNKQRTVVPARCGVTVRDSLKKALMMRGLIPECCAVYRIQDGEKKPIGWDTDISWLTGEELHVEVLENVPLTTHNFVRKTFFTLAFCDFCRKLLFQGFRCQTCGYKFHQRCSTEVPLMCVNYDQLDLLFVSKFFEHHPIPQEEASLAETTLPCGSSPSAPPSDSIGPPILTSPSPSKSIPIPQPFRPADEDHRNQFGQRDRSSSAPNVHINTIEPVNIDDLIRDQGFRSDGGSTTGLSATPPASLPGSLSNVKALQKSPGPQRERKSSSSSEDRNRMKTLGRRDSSDDWEIPDGQITVGQRIGSGSFGTVYKGKWHGDVAVKMLNVTAPTPQQLQAFKNEVGVLRKTRHVNILLFMGYSTKPQLAIVTQWCEGSSLYHHLHIIETKFEMIKLIDIARQTAQGMDYLHAKSIIHRDLKSNNIFLHEDLTVKIGDFGLATVKSRWSGSHQFEQLSGSILWMAPEVIRMQDKNPYSFQSDVYAFGIVLYELMTGQLPYSNINNRDQVLCPPWECNKCCARAYFP

SEQ ID NO: 35 - DNA, 2319 bp, Bos taurus
ctcagctgcgccgggtctcacaagacggttcccgaggtggcccaggcgccgtcccaccgccgacgccgcccgggccgcccgggccgtccctccccgctgccccccgtcctccgcctccgcctccccccgccctcagcctcccttccccctccccgcccagcagcggtcgctcgggcccggctctcggttataagatggcggcgctgagtggcggcggcggcggcggcggcggtggcgcggagcagggccaggctctgttcaacggggacatggagcccgaggccggcgccgcggcctcttcggctgcggaccccgccattcccgaggaggtgtggaatatcaaacaaatgattaagttgacacaggagcatatagaggccctattggacaaatttggtggggagcataatccaccatcaatatatctggaggcctatgaagaatacaccagcaagctagatgccctccaacaaagagaacaacagttattggaatccctggggaatggaactgatttttctgtttctagctctgcatcaacggacaccgttacatcttcttcctcttctagcctttcagtgctgccttcatctctttcagtttttcaaaatcccacagatgtgtcacggagcaaccccaagtcaccacaaaaacctatcgttagagtcttcctgcccaataaacagaggacagtggtacctgcacggtgtggagtcacagtccgggacagcctgaagaaggcactgatgatgagaggtctaatcccagagtgctgtgctgtttacagaattcaggatggggagaagaaaccaattggctgggacactgatatttcctggcttactggagaggagttgcatgtagaagtgttggagaatgttccacttacaacacacaactttgtacggaaaacttttttcaccttagcattttgtgacttctgtagaaagctgcttttccagggattccgctgtcaaacatgtggttataaatttcaccagcgttgtagtacagaggttccactgatgtgtgttaattatgaccaactagatttgctgtttgtctccaagttctttgaacaccacccaataccacaggaggaggcctccttagcagagactacccttccatgtggctcatccccttctgcacccccctccgattctattgggcccccaattctcaccagtccatctccttcaaaatccattccaattccacagcctttccgaccagcagatgaagatcatcgaaatcagtttggacaacgagaccggtcctcatcagctccaaatgtgcatataaacacaatagaacccgtcaatattgatgacttgattagagaccaagggtttcgtagtgatggaggatcaaccacaggtttatccgccacaccccctgcctcattacctggctcactctctaatgtgaaagcattgcagaaatctccaggacctcagcgagaaagaaagtcctcttcatcctcagaagacaggaatcgaatgaaaacgcttggtagacgggattcaagtgacgattgggagattcctgatggacagatcacagtgggacaaagaattggatcagggtcatttgggacagtctacaagggaaagtggcatggtgatgtggcagtgaaaatgttgaatgtgacagcacccacacctcagcagttacaggccttcaaaaatgaagtaggagtactcaggaaaacgcgacatgtgaatatcctcctcttcatgggttattcaacaaagccacaactggctattgttacccagtggtgtgagggctccagtttatatcatcatctccacatcattgagaccaaattcgagatgatcaaacttatagatattgcacggcagactgcacagggcatggattacttacacgccaagtcaatcatccacagagacctcaagagtaataatatttttcttcatgaagacctcacagtaaaaataggtgattttggtctagccacagtgaaatctcgatggagtgggtcccatcagtttgaacagttgtctggatccattttgtggatggcaccagaagtaatcagaatgcaagataaaaacccatatagctttcagtcagatgtatatgcatttgggattgttctgtatgaattgatgaccggacagttaccttattcaaatatcaacaacagggaccaggtgctttgtcctccatgggagtgtaataaatgctgtgcaagggcttacttcccatgagagaagtgagtgaccaacagaaggtctgtgcaaggaaaagagacaaagccacggatcagaagcacatggccataactga

SEQ ID NO: 36 - protein, 681 aa, Bos taurus; identical to SEQ ID NO: 34

SEQ ID NO: 37 - DNA, 2661 bp, Bos taurus
tcagctgcgccgggtctcacaagacggttcccgaggtggcccaggcgccgtcccaccgccgacgccgcccgggccgcccgggccgtccctccccgctgccccccgtcctccgcctccgcctccccccgccctcagcctcccttccccctccccgcccagcagcggtcgctcgggcccggctctcggttataagatggcggcgctgagtggcggcggcggcggcggcggcggtggcgcggagcagggccaggctctgttcaacggggacatggagcccgaggccggcgccgcggcctcttcggctgcggaccccgccattcccgaggaggtgtggaatatcaaacaaatgattaagttgacacaggagcatatagaggccctattggacaaatttggtggggagcataatccaccatcaatatatctggaggcctatgaagaatacaccagcaagctagatgccctccaacaaagagaacaacagttattggaatccctggggaatggaactgatttttctgtttctagctctgcatcaacggacaccgttacatcttcttcctcttctagcctttcagtgctgccttcatctctttcagtttttcaaaatcccacagatgtgtcacggagcaaccccaagtcaccacaaaaacctatcgttagagtcttcctgcccaataaacagaggacagtggtacctgcacggtgtggagtcacagtccgggacagcctgaagaaggcactgatgatgagaggtctaatcccagagtgctgtgctgtttacagaattcaggatggggagaagaaaccaattggctgggacactgatatttcctggcttactggagaggagttgcatgtagaagtgttggagaatgttccacttacaacacacaactttgtacggaaaacttttttcaccttagcattttgtgacttctgtagaaagctgcttttccagggattccgctgtcaaacatgtggttataaatttcaccagcgttgtagtacagaggttccactgatgtgtgttaattatgaccaactagatttgctgtttgtctccaagttctttgaacaccacccaataccacaggaggaggcctccttagcagagactacccttccatgtggctcatccccttctgcacccccctccgattctattgggcccccaattctcaccagtccatctccttcaaaatccattccaattccacagcctttccgaccagcagatgaagatcatcgaaatcagtttggacaacgagaccggtcctcatcagctccaaatgtgcatataaacacaatagaacccgtcaatattgatgacttgattagagaccaagggtttcgtagtgatggaggatcaaccacaggtttatccgccacaccccctgcctcattacctggctcactctctaatgtgaaagcattgcagaaatctccaggacctcagcgagaaagaaagtcctcttcatcctcagaagacaggaatcgaatgaaaacgcttggtagacgggattcaagtgacgattgggagattcctgatggacagatcacagtgggacaaagaattggatcagggtcatttgggacagtctacaagggaaagtggcatggtgatgtggcagtgaaaatgttgaatgtgacagcacccacacctcagcagttacaggccttcaaaaatgaagtaggagtactcaggaaaacgcgacatgtgaatatcctcctcttcatgggttattcaacaaagccacaactggctattgttacccagtggtgtgagggctccagtttatatcatcatctccacatcattgagaccaaattcgagatgatcaaacttatagatattgcacggcagactgcacagggcatggattacttacacgccaagtcaatcatccacagagacctcaagagtaataatatttttcttcatgaagacctcacagtaaaaataggtgattttggtctagccacagtgaaatctcgatggagtgggtcccatcagtttgaacagttgtctggatccattttgtggatggcaccagaagtaatcagaatgcaagataaaaacccatatagctttcagtcagatgtatatgcatttgggattgttctgtatgaattgatgaccggacagttaccttattcaaatatcaacaacagggaccagtctgtgcaaggaaaagagacaaagccacggatcagaagcacatggccataactgaagattttgtgaactctcacaaggaaaaaatttgctctttgaacaataagaaggaactcactaaaatgtaactgagaactgttcaacaggttgaaagctgaaagatgccattggaactgacaaaatgtttcttaaacataaatgatgaaacagtgaaactacataatatctcctctggctgaaacattcaagaagtttaaaatgcttaagttaaaaataaaatcctagtaaacaatggacttactgtgcaacatagagaatatcttacgataacctgtaatggaaaagaatctgaaaaagaatgtatataactgaatcactttgctgtaaactagaatctgacacaacactgtaaatcactacacttttctgttgcatgccaaagattatttaataacgtcattaaaaaattattttaataatta

SEQ ID NO: 38 - protein, 679 aa, Bos taurus
MAALSGGGGGGGGGAEQGQALFNGDMEPEAGAAASSAADPAIPEEVWNIKQMIKLTQEHIEALLDKFGGEHNPPSIYLEAYEEYTSKLDALQQREQQLLESLGNGTDFSVSSSASTDTVTSSSSSSLSVLPSSLSVFQNPTDVSRSNPKSPQKPIVRVFLPNKQRTVVPARCGVTVRDSLKKALMMRGLIPECCAVYRIQDGEKKPIGWDTDISWLTGEELHVEVLENVPLTTHNFVRKTFFTLAFCDFCRKLLFQGFRCQTCGYKFHQRCSTEVPLMCVNYDQLDLLFVSKFFEHHPIPQEEASLAETTLPCGSSPSAPPSDSIGPPILTSPSPSKSIPIPQPFRPADEDHRNQFGQRDRSSSAPNVHINTIEPVNIDDLIRDQGFRSDGGSTTGLSATPPASLPGSLSNVKALQKSPGPQRERKSSSSSEDRNRMKTLGRRDSSDDWEIPDGQITVGQRIGSGSFGTVYKGKWHGDVAVKMLNVTAPTPQQLQAFKNEVGVLRKTRHVNILLFMGYSTKPQLAIVTQWCEGSSLYHHLHIIETKFEMIKLIDIARQTAQGMDYLHAKSIIHRDLKSNNIFLHEDLTVKIGDFGLATVKSRWSGSHQFEQLSGSILWMAPEVIRMQDKNPYSFQSDVYAFGIVLYELMTGQLPYSNINNRDQSVQGKETKPRIRSTWP

SEQ ID NO: 39 - DNA, 7434 bp, Bos taurus
acaccgttacatcttcttcctcttctagcctttcagtgctgccttcatctctttcagtttttcaaaatcccacagatgtgtcacggagcaaccccaagtcaccacaaaaacctatcgttagagtcttcctgcccaataaacagaggacagtggtacctgcacggtgtggagtcacagtccgggacagcctgaagaaggcactgatgatgagaggtctaatcccagagtgctgtgctgtttacagaattcaggatggggagaagaaaccaattggctgggacactgatatttcctggcttactggagaggagttgcatgtagaagtgttggagaatgttccacttacaacacacaactttgtacggaaaacttttttcaccttagcattttgtgacttctgtagaaagctgcttttccagggattccgctgtcaaacatgtggttataaatttcaccagcgttgtagtacagaggttccactgatgtgtgttaattatgaccaactagatttgctgtttgtctccaagttctttgaacaccacccaataccacaggaggaggcctccttagcagagactacccttccatgtggctcatccccttctgcacccccctccgattctattgggcccccaattctcaccagtccatctccttcaaaatccattccaattccacagcctttccgaccagcagatgaagatcatcgaaatcagtttggacaacgagaccggtcctcatcagctccaaatgtgcatataaacacaatagaacccgtcaatattgatgacttgattagagaccaagggtttcgtagtgatggaggatcaaccacaggtttatccgccacaccccctgcctcattacctggctcactctctaatgtgaaagcattgcagaaatctccaggacctcagcgagaaagaaagtcctcttcatcctcagaagacaggaatcgaatgaaaacgcttggtagacgggattcaagtgacgattgggagattcctgatggacagatcacagtgggacaaagaattggatcagggtcatttgggacagtctacaagggaaagtggcatggtgatgtggcagtgaaaatgttgaatgtgacagcacccacacctcagcagttacaggccttcaaaaatgaagtaggagtactcaggaaaacgcgacatgtgaatatcctcctcttcatgggttattcaacaaagccacaactggctattgttacccagtggtgtgagggctccagtttatatcatcatctccacatcattgagaccaaattcgagatgatcaaacttatagatattgcacggcagactgcacagggcatggattacttacacgccaagtcaatcatccacagagacctcaagagtaataatatttttcttcatgaagacctcacagtaaaaataggtgattttggtctagccacagtgaaatctcgatggagtgggtcccatcagtttgaacagttgtctggatccattttgtggatggcaccagaagtaatcagaatgcaagataaaaacccatatagctttcagtcagatgtatatgcatttgggattgttctgtatgaattgatgaccggacagttaccttattcaaatatcaacaacagggaccagataatttttatggtgggacgaggatatctgtctccagatctcagtaaggtacggagtaactgtccaaaagccatgaagagattaatggcagagtgcctaaaaaagaaaagagatgaaagaccactctttccccaagtaggaaagactctcctaagcaagagacaaaattcagaagttatcagggaaaaagataagcagattctcgcctctattgagctgctggcccgctcattgccaaaaattcaccgcagtgcatcagaaccctccttgaatcgggctggcttccaaacagaggattttagtctatatgcttgtgcttctccaaaaacacccattcaggcagggggatatggagaatttgcagccttcaagtagccacaccatcatgacagcatctactcttatttcttaagtcttgtgttcgtacaatttgttaacatcaaaacacagttctgttcctcaactctttttaaagttaaaatttttcagtgcataagctggtgtggaacagaaggaaatttcccatccaacaaaagagggaagaatgttttaggaaccagaattctctgctgccagtgtttcttcttcaacacaaatatcacaagtctgcccactcccaggaagaaagaggagagaccctgagttctgaccttttgatggtcaggcatgatggaaagaaactgctgctacagcttgggagatttgctctgggaagtctgccagtcaactttgcccttctaaccaccagatcaatatgtggctgatcatctgatggggcagttgcaatcaccaagccttgttctctttcctgttctgggattgtgttgtggaacccttttccctagccaccaccagttcatttctgagggatggaacaaaaatgcagcatgcccttcctgtgtggtgcatgttcagtccttgacaaatttttaccaaaatgaagctactttatttaaaaggagggtgagaggtgaggaggtcactttgggtgtggcggaaagggaatgctgcatctttttcctgggctgctggggctctggccttggcttgccagccggaagcgctggcacgcatcgccttcttttcccattgggtccagcaatgaagacgagtgtttggggttttttttttctccaccatgtagcaagttctcaggaaaatacaattgatatcttcctcctaagctcttccaatcagtcaccaagtacttatgtggttactttgtccagggcacaaaatgcctgtatctaattaaaagcctacaaaactgcttgataacagttttgaatgtgagacatttatgtaatttaaatgtaaggtacaagttttaatttctgagtttcttctattatatttttattaaaaaaagaaaataattttcagattgaattggagtaaaataatattacttcccactagaattatatatcctggaaaattgtatttttgttacataagcagcttttaaagaaagatcattacccttttctctacataaatatatggggagtcttagcctaatgacaaatatttataatttttaaattaatggtacttgctggatccatactaacatctttactaatacctcattgtttcttccaacttactcctacactacatcctacatcttcttcctagtcttttatctagaatatgcaacctcaaataaaaatggtggtgtcctcattcattctcctccttccttttttcccaagcctgatcttcaaaaggttggttaatttggcagctgagttcctccccaggcagagaatagaccaattttaggtgtattgggactgagggaggatgtgtaaagattaacatcagtaaagaaccgctgtggagtaattaagaactttgttctttataactggagaatataacctaaccctaacatccctcagcctttactaaagtgtggcgtaaatcacagtagtagcaaagaaagtgactctggatgtgttcctggccagtacctcccttatcatgaatgtagactctctcatcaagatttaggaatataaatcaaatcaaatgtgcccagccaagctatgtagtaagggacttgaacaatattaggcagaacctataaaataaatcagggaattagaaattatttaaagttttcaaattgtaaattgccccggtgtctttcagcctactgccattatttttgctacaatacctacatttcagaggagggcctactgaaaattccatgcaagtggaaaataatcctcaagttattaatgagtttgaaaagcaatgagttcttaagtctttgtgagtagagcaagatcctacaaaattcagaaatagtaaaaatggattcatgctgatttgaagagcatctgtgtgcataatataatgctgcatctcttttaaaagcagtctatttttctttttaaatttgtccccatagatgcttttgaacatgaacatgcttatgttaccttttccgaggttgggaagagccaggagctctcaggcagggccccctccctcagctgggcaggagctgctcaggaggagctagttatagaggaagcttagcgttggcattttcaaaattcaaggtgataacgctttcttcttcctttctgttttagaatagattgctgtctgatttgaaaaagggaaatagatttgatctcaaatgaatctgtgcccagaagccaggctcagggtattcagagatttgtatagtgccctcaaaaaataacaaaattttagctttccttttttcttcttttctccatcaaattcttttttctctagtttacaaatgacatggaaaaggaatttcccctgagttttgtatgcctttttttttttggcttagactatagataggcgtgttgagctcctaagaaaatacaaggaggaactctttgttgtgcagagcactttatgagtagtttgtgtggataatatgtgactgcttccctgacgagcttgtgaggctgtacttatgtctttcctgtaaggcagcttcagtgccttctgtagtgtatataaggaaagattacgccttctgaaaaatctcagagcaaccataagattattttaaaatatgtagtatgactgatggactttttcatcattaaattagtctagcatctaaacttttaccactgaaataatattgaccaaaaagcaatttataaaaggtatttgtgaatagaaaatacaatgtgatcatttgtacttatgtgcaccttaaaagaggaattctgtctagctgtcaaattctggttccttaacatccagtccttgattgtgattgagatctggtaggacgtgctggggcacgctagcagataaaatcccgtatactttaggatagatgttacatttatgtcagtgttggcaaagagcattgtgtagtaataaagaattcaagacttcagcaatgtcaacctgaaactttgtaaatatttcctagattgttatttgatgcagtcacagctctttatcacacaatgttgtctttccctcatcaggcaattttagaactgctgcacacccctcctcagatctcacctgcccctcctgtacattcacctctccagccttgtgcacacctcatttagctttagtttgaaacacattgcagggttcaggtgacctcttcaaaaactacctcctcagaatgaggtaatgaatagttatttattttaaaatatgaaaagtcaggagctctagaatatgaagatgatctaagattttaacttttatgtatacttgttgagcactctccttttgtcctaaagggcattatacatttaagcagtaatactgaaaaatgtagctcagagtaactgaatgttgttgaaagtggtgccagaatctgttttaggggtacgtatcagaatcttaatcttaaatcggttacatgaaattaaatagttaatggtaacacttgactaacagatataattttaattttcggtaggcttttagcaagacagtaagtacatcttcataatgagttagccacagcttcatcacatgcacagattttcctgttgagagactgcccagttaagagggtagaatgatgaaccatttttcaggattctcttctttgtccaaactggcattgtgagtgctagaatatcagcactttcaaactagtgattccaactattaggctattaaaaagcaaaacaaaccaaacaaaccatagccagacatgggaagtttactatgagtataaacagcaaatagcttacaggtcatacattgaaatggtgtaggtaaggcgttagaaaaataccttgacaatttgccaaatgatcttactgtgccttcatgatgcaataaaaaaaaaaaaaatttagcataaatcagtgatttgtgaagagagcagccaccctggtctaactcagctgtgttaatattttttagcgtgcaatttagactgcaaagataaatgcactaaagagtttatagccaaaatcacatttaaaaaatgagagaaaacacaggtaaattttcagtgaacaaaattatttttttaaagtacataatccctagtatagtcagatatatttatcacatagagcaaataggttgaaatcacaattcagtgacatttctagagaaactttttctactcccataggttcttcaaagcatggaacttttatataacagaaatgtgtgacggtcattttaaattgctgtagtttggggctgaagtactgtgtgctgggcagcaatcacatgtattaactagtgagaaaggagaaattaagatataggacagaatttgattttcttgttcccagattactgctgccaacctagacactgagtttccagaggctgaaacgtaaacttgcagctcagcaactgttttgcaaagttagtgggactgtcctgcttatgctgttcaaaaatgctctgagggccaggtggggcctccaggggctcctctctgaggggacatcagactagctaacgacctggcgggcggatgtgaaccggacacactccatggtgtgcttcttgtatcggtccctcgccaccctcaagaaaggcttcagcgggttctctagacgtctccactaaggtgtgttactaacagccatgggttgttgagcacccgaggagtgcaatagcatctctgcatgattgtatattggcccgaagagaatgaagtggccagtgtactcatgttccatgttgctagctctggtaaactgaaaatactggtaagatttttgttttatcagtacactagagagtaagctttgttttgttgtttttagataatgttttcacttccatttggaaagacatttaaattgagtttcagtcctaaattttgccagtcatggtaattagcagtttctatcaggtatttttaaggtagaagaggatagaaacataagttctaaaagcttaaggtaaccgtggtttattttaaaatgtttaggggtggttagtctctacctcaaaaaaagtgagtgaatcttttatttcagcattcacaagttcggctgttgtttttgtaatacattttttttttaaccttttgacccccctttacctaagtgtcaatgtagttttattaattactaagtcagtttcattaaaatgtttatttagcagttttgactaattgcaatgattaatatagccagttgtgcatgaggacacagccagtgagtatatctgggttttttttgtgatgctttttttcttaagacttctgtagatttatgaagtactcattgaaaacaactaaaatacgtttattcgtgttaatatggaaaaaaaaaaa

SEQ ID NO: 40 - protein, 603 aa, Bos taurus
MMRGLIPECCAVYRIQDGEKKPIGWDTDISWLTGEELHVEVLENVPLTTHNFVRKTFFTLAFCDFCRKLLFQGFRCQTCGYKFHQRCSTEVPLMCVNYDQLDLLFVSKFFEHHPIPQEEASLAETTLPCGSSPSAPPSDSIGPPILTSPSPSKSIPIPQPFRPADEDHRNQFGQRDRSSSAPNVHINTIEPVNIDDLIRDQGFRSDGGSTTGLSATPPASLPGSLSNVKALQKSPGPQRERKSSSSSEDRNRMKTLGRRDSSDDWEIPDGQITVGQRIGSGSFGTVYKGKWHGDVAVKMLNVTAPTPQQLQAFKNEVGVLRKTRHVNILLFMGYSTKPQLAIVTQWCEGSSLYHHLHIIETKFEMIKLIDIARQTAQGMDYLHAKSIIHRDLKSNNIFLHEDLTVKIGDFGLATVKSRWSGSHQFEQLSGSILWMAPEVIRMQDKNPYSFQSDVYAFGIVLYELMTGQLPYSNINNRDQIIFMVGRGYLSPDLSKVRSNCPKAMKRLMAECLKKKRDERPLFPQVGKTLLSKRQNSEVIREKDKQILASIELLARSLPKIHRSASEPSLNRAGFQTEDFSLYACASPKTPIQAGGYGEFAAFK

SEQ ID NO: 41 - DNA, 2295 bp, Equus caballus
  misc_feature (79)..(79): n is a, c, g, or t
atgaagacgctgagcggcggcggcggcggcgcggagcagggccaggctctgttcaacggggacatggaacccggaggcnccgcgccggcgcccgcggcctcgtcggccgcggaccctgccattcccgaggaggtatggaatatcaaacaaatgattaaattgacacaggaacatatagaggccctattggacaaatttggtggggagcataatccaccatcaatatatctggaggcctatgaagaatacaccagcaagctagatgccctccaacaaagagaacaacagttattggaatccctggggaatggaactgatttttctgtttctagttctgcatcaacggacaccgttacatcttcttcctcttctagcctttcagtgctaccttcatctctttcagtttttcaaaatcccacagatgtgtcacggagcaaccctaagtcaccacaaaaacctatcgttagagtcttcctgcccaacaaacagaggacagtggtacctgcaaggtgtggcgttacagtccgggacagtctaaagaaagcactgatgatgagaggtctaatcccagagtgctgtgctgtttacagaattcaggatggagagaagaaaccaattggctgggacactgatatttcctggctcactggagaggaattgcatgtagaagtgttggagaatgttccacttacaacacacaactttgtacggaaaacttttttcaccttagcattttgtgacttttgtcgaaagctgcttttccagggtttccgctgtcaaacatgtggttataaatttcaccagcgttgtagtacagaggttccactgatgtgtgttaattatgaccaacttgatttgctgtttgtctccaagttctttgaacaccacccagtatcacaggaggaggcctccttagcagagactgcccttacatctggatcatccccttctgcacccccctccgattccattgggccccaaattctcaccagtccatctccttcaaaatccattccaattccacagcctttccgaccagcagatgaagatcatcgaaatcagtttggacaacgagaccggtcctcatcagctccaaatgtacatataaacacaatagaacctgtcaatattgatgacttgattagagaccaagggtttcgtagtgatggaggatcaaccacaggtttatctgccaccccccctgcctcattacctggctcactcactaatgtgaaggcattacagaaatctccaggacctcaacgggaaaggaaatcatcttcatcctcagaagacaggaatcgaatgaaaactcttggtagacgggattcaagtgacgattgggagattcctgatgggcagatcacagtgggacaaagaattggatctgggtcatttgggacagtctacaagggaaagtggcatggtgatgtggcagtgaaaatgttgaatgtgacagcacccacacctcagcagttacaggccttcaaaaatgaagtaggagtactcaggaaaactcgacatgtgaatatcctactcttcatgggctattcaacaaagccacaactggctattgttacccagtggtgtgagggctccagcttatatcaccatctccacatcattgagaccaaatttgagatgatcaaacttatagatattgctcggcaaactgcacagggcatggattacttacacgccaagtcaatcatccacagagacctcaagagtaataatatttttcttcatgaagacctcacagtaaaaataggtgattttggtctagccacagtgaaatctcgatggagtgggtcccatcagtttgaacagttgtctggatccattttgtggatggcaccagaagtaatcagaatgcaagataaaaacccgtatagctttcaatcagatgtatatgcctttgggattgttctgtatgaattgatgactggacagttaccttattcaaacatcaacaacagggaccagataatttttatggtgggaagaggatatctatctccagatctcagtaaggtacggagtaactgtccaaaagccatgaagagattaatggcagagtgcctaaaaaagaaaagagacgagagaccactcttcccccaaattctcgcctctattgagctgctggcccgctcattgccaaaaattcaccgcagtgcatcagagccctccttgaatcgggctggcttccagacagaggattttagtctatatgcttgtgcttctccgaaaacacccatccaggcagggggatatggtgcgtttcctgtccactga

SEQ ID NO: 42 - protein, 764 aa, Equus caballus
  misc_feature (27)..(27): Xaa can be any naturally occurring amino acid
MKTLSGGGGGAEQGQALFNGDMEPGGXAPAPAASSAADPAIPEEVWNIKQMIKLTQEHIEALLDKFGGEHNPPSIYLEAYEEYTSKLDALQQREQQLLESLGNGTDFSVSSSASTDTVTSSSSSSLSVLPSSLSVFQNPTDVSRSNPKSPQKPIVRVFLPNKQRTVVPARCGVTVRDSLKKALMMRGLIPECCAVYRIQDGEKKPIGWDTDISWLTGEELHVEVLENVPLTTHNFVRKTFFTLAFCDFCRKLLFQGFRCQTCGYKFHQRCSTEVPLMCVNYDQLDLLFVSKFFEHHPVSQEEASLAETALTSGSSPSAPPSDSIGPQILTSPSPSKSIPIPQPFRPADEDHRNQFGQRDRSSSAPNVHINTIEPVNIDDLIRDQGFRSDGGSTTGLSATPPASLPGSLTNVKALQKSPGPQRERKSSSSSEDRNRMKTLGRRDSSDDWEIPDGQITVGQRIGSGSFGTVYKGKWHGDVAVKMLNVTAPTPQQLQAFKNEVGVLRKTRHVNILLFMGYSTKPQLAIVTQWCEGSSLYHHLHIIETKFEMIKLIDIARQTAQGMDYLHAKSIIHRDLKSNNIFLHEDLTVKIGDFGLATVKSRWSGSHQFEQLSGSILWMAPEVIRMQDKNPYSFQSDVYAFGIVLYELMTGQLPYSNINNRDQIIFMVGRGYLSPDLSKVRSNCPKAMKRLMAECLKKKRDERPLFPQILASIELLARSLPKIHRSASEPSLNRAGFQTEDFSLYACASPKTPIQAGGYGAFPVH

SEQ ID NO: 43 - DNA, 2678 bp, Gallus gallus
tccccctccctcgccccagcgcttcgatccaagatggcggcgctgagcagcggcagcagcgccgagggggcctcgctcttcaacggggacatggagcccgagccgccgccgcccgtgctgggcgcctgctacgccgggagcggcggcggcgacccggccatcccggaggaggtgtggaatatcaaacagatgattaaattaacacaagaacatatagaagcgctgttagacaagtttggaggagagcataacccaccatcaatatatttagaggcctatgaggagtacaccagcaaactagatgctctacagcagagagaacagcagttattggaatccatgggaaatggaactgatttctctgtttccagttcagcttcaacggacacagttgcatcatcttcctcctctagcctctctgtagcaccttcatccctttcagtttatcaaaatcctactgatatgtcgcggaataaccctaagtctccacagaagcctattgttagagtcttcctgcccaacaagcaaaggactgtggttccggcaagatgtggggtgacagtccgagacagcctgaagaaagctctgatgatgagaggtcttattccagaatgctgtgctgtttacagaatacaggatggagagaagaagccaattggctgggacactgacatttcctggctaaccggagaggagttacacgtggaggtcttggagaatgtgccactcacaacacacaattttgtacgaaaaacattcttcacgttagcgttctgcgacttctgtcgaaagctgcttttccagggattccgatgccagacatgtggctacaaatttcaccagcgctgtagcacagaagtgccactgatgtgtgttaactacgaccaactcgatttgctgtttgtctccaagttctttgaacatcaccccatatcgcaggaggagaccaccttaggagagaccaccccggcatcgggatcgtacccctcagtgcccccatcagattctgttggaccaccaattctccctagtccttctccttcaaaatccattccaatcccacagcccttccgaccagcagatgaagaccatcggaatcagtttgggcaacgcgaccgatcctcttcagctcccaatgttcacatcaatacaattgagccagtcaatattgatgacttgattagagaccagggtgtacgaggagagggagcccctttgaaccagctgatgcgctgtcttcggaaataccaatcccggactcccagtcccctccttcattctgtccccagtgaaatagtgtttgattttgagcctggcccagtgttcagaggttcaactgcaggtttgtctgcaacacctcctgcatctttgcctgggtcacttaccaatgtgaaagcattacagaaatcaccaggcccccaacgggaaaggaaatcatcctcatcctcagaagacagaaataggatgaaaacccttggtcgacgagattcaagtgatgattgggaaataccagatgggcagatcacagttggacaaaggataggatctggatcatttggaacagtctacaaaggaaagtggcatggtgacgtggcagtgaaaatgttgaatgttacagcacccacacctcaacagttacaggctttcaaaaatgaagtaggagtgctcaggaaaacacggcatgtgaatatcctactttttatgggttattcaacaaaacctcagttggctattgttacacagtggtgtgaggggtccagcttatatcaccatctgcacataattgagaccaagtttgaaatgatcaaactaattgatattgcacgacagactgcacaaggcatggattatttgcatgccaagtcaatcatccacagagacctcaagagtaataatatttttcttcatgaagacctcacagtaaaaataggtgacttcggtctggctacagtgaaatcacgatggagtggatctcatcaatttgaacagttatctggatcaattctatggatggcaccggaagtgatcaggatgcaagacaaaaacccatatagctttcagtcagatgtgtatgcattcgggattgtgctttatgaactgatgactggacagttaccatactcaaacatcaacaacagggaccagataatttttatggtgggacgaggatatctatctccagacctcagtaaagtaagaagtaactgtccaaaagctatgaagagactaatggcagaatgcttgaaaaagaaaagagatgagagacctctttttccacagattcttgcctccattgagcttctggcccggtcgttgccaaaaattcaccgcagtgcatctgagccgtcactaaaccgggctggcttccagaccgaggatttcagtctgtatgcttgtgcttctccaaaaacgcccatccaagcagggggatacggtgggtttccagtacactgaaaagaaatgtgaaagcgtgtgcctgtttgctcatgtgctggtgtgttcctgtgtgtgcaacgcatacgtacgttctcagttcctaccagcgactttttaaggtttactgagggaatgaagactcatttcctaacatggggcattgaacgtcctgagcacaagtcagtgctggtaaggaatgtcttgggaacagctggcaagaagaattagaaggtacttaaagg

SEQ ID NO: 44 - protein, 806 aa, Gallus gallus
MAALSSGSSAEGASLFNGDMEPEPPPPVLGACYAGSGGGDPAIPEEVWNIKQMIKLTQEHIEALLDKFGGEHNPPSIYLEAYEEYTSKLDALQQREQQLLESMGNGTDFSVSSSASTDTVASSSSSSLSVAPSSLSVYQNPTDMSRNNPKSPQKPIVRVFLPNKQRTVVPARCGVTVRDSLKKALMMRGLIPECCAVYRIQDGEKKPIGWDTDISWLTGEELHVEVLENVPLTTHNFVRKTFFTLAFCDFCRKLLFQGFRCQTCGYKFHQRCSTEVPLMCVNYDQLDLLFVSKFFEHHPISQEETTLGETTPASGSYPSVPPSDSVGPPILPSPSPSKSIPIPQPFRPADEDHRNQFGQRDRSSSAPNVHINTIEPVNIDDLIRDQGVRGEGAPLNQLMRCLRKYQSRTPSPLLHSVPSEIVFDFEPGPVFRGSTAGLSATPPASLPGSLTNVKALQKSPGPQRERKSSSSSEDRNRMKTLGRRDSSDDWEIPDGQITVGQRIGSGSFGTVYKGKWHGDVAVKMLNVTAPTPQQLQAFKNEVGVLRKTRHVNILLFMGYSTKPQLAIVTQWCEGSSLYHHLHIIETKFEMIKLIDIARQTAQGMDYLHAKSIIHRDLKSNNIFLHEDLTVKIGDFGLATVKSRWSGSHQFEQLSGSILWMAPEVIRMQDKNPYSFQSDVYAFGIVLYELMTGQLPYSNINNRDQIIFMVGRGYLSPDLSKVRSNCPKAMKRLMAECLKKKRDERPLFPQILASIELLARSLPKIHRSASEPSLNRAGFQTEDFSLYACASPKTPIQAGGYGGFPVH

SEQ ID NO: 45 - DNA, 2949 bp, Homo sapiens
cgcctcccttccccctccccgcccgacagcggccgctcgggccccggctctcggttataagatggcggcgctgagcggtggcggtggtggcggcgcggagccgggccaggctctgttcaacggggacatggagcccgaggccggcgccggcgccggcgccgcggcctcttcggctgcggaccctgccattccggaggaggtgtggaatatcaaacaaatgattaagttgacacaggaacatatagaggccctattggacaaatttggtggggagcataatccaccatcaatatatctggaggcctatgaagaatacaccagcaagctagatgcactccaacaaagagaacaacagttattggaatctctggggaacggaactgatttttctgtttctagctctgcatcaatggataccgttacatcttcttcctcttctagcctttcagtgctaccttcatctctttcagtttttcaaaatcccacagatgtggcacggagcaaccccaagtcaccacaaaaacctatcgttagagtcttcctgcccaacaaacagaggacagtggtacctgcaaggtgtggagttacagtccgagacagtctaaagaaagcactgatgatgagaggtctaatcccagagtgctgtgctgtttacagaattcaggatggagagaagaaaccaattggttgggacactgatatttcctggcttactggagaagaattgcatgtggaagtgttggagaatgttccacttacaacacacaactttgtacgaaaaacgtttttcaccttagcattttgtgacttttgtcgaaagctgcttttccagggtttccgctgtcaaacatgtggttataaatttcaccagcgttgtagtacagaagttccactgatgtgtgttaattatgaccaacttgatttgctgtttgtctccaagttctttgaacaccacccaataccacaggaagaggcgtccttagcagagactgccctaacatctggatcatccccttccgcacccgcctcggactctattgggccccaaattctcaccagtccgtctccttcaaaatccattccaattccacagcccttccgaccagcagatgaagatcatcgaaatcaatttgggcaacgagaccgatcctcatcagctcccaatgtgcatataaacacaatagaacctgtcaatattgatgacttgattagagaccaaggatttcgtggtgatggaggatcaaccacaggtttgtctgctaccccccctgcctcattacctggctcactaactaacgtgaaagccttacagaaatctccaggacctcagcgagaaaggaagtcatcttcatcctcagaagacaggaatcgaatgaaaacacttggtagacgggactcgagtgatgattgggagattcctgatgggcagattacagtgggacaaagaattggatctggatcatttggaacagtctacaagggaaagtggcatggtgatgtggcagtgaaaatgttgaatgtgacagcacctacacctcagcagttacaagccttcaaaaatgaagtaggagtactcaggaaaacacgacatgtgaatatcctactcttcatgggctattccacaaagccacaactggctattgttacccagtggtgtgagggctccagcttgtatcaccatctccatatcattgagaccaaatttgagatgatcaaacttatagatattgcacgacagactgcacagggcatggattacttacacgccaagtcaatcatccacagagacctcaagagtaataatatatttcttcatgaagacctcacagtaaaaataggtgattttggtctagctacagagaaatctcgatggagtgggtcccatcagtttgaacagttgtctggatccattttgtggatggcaccagaagtcatcagaatgcaagataaaaatccatacagctttcagtcagatgtatatgcatttggaattgttctgtatgaattgatgactggacagttaccttattcaaacatcaacaacagggaccagataatttttatggtgggacgaggatacctgtctccagatctcagtaaggtacggagtaactgtccaaaagccatgaagagattaatggcagagtgcctcaaaaagaaaagagatgagagaccactctttccccaaattctcgcctctattgagctgctggcccgctcattgccaaaaattcaccgcagtgcatcagaaccctccttgaatcgggctggtttccaaacagaggattttagtctatatgcttgtgcttctccaaaaacacccatccaggcagggggatatggtgcgtttcctgtccactgaaacaaatgagtgagagagttcaggagagtagcaacaaaaggaaaataaatgaacatatgtttgcttatatgttaaattgaataaaatactctctttttttttaaggtgaaccaaagaacacttgtgtggttaaagactagatataatttttccccaaactaaaatttatacttaacattggatttttaacatccaagggttaaaatacatagacattgctaaaaattggcagagcctcttctagaggctttactttctgttccgggtttgtatcattcacttggttattttaagtagtaaacttcagtttctcatgcaacttttgttgccagctatcacatgtccactagggactccagaagaagaccctacctatgcctgtgtttgcaggtgagaagttggcagtcggttagcctgggttagataaggcaaactgaacagatctaatttaggaagtcagtagaatttaataattctattattattcttaataatttttctataactatttctttttataacaatttggaaaatgtggatgtcttttatttccttgaagcaataaactaagtttctttttataaaaa

SEQ ID NO: 46 - DNA, 21 bp, Artificial Sequence
  BRAF siRNA 313
tacaccagcaagctagatgca

SEQ ID NO: 47 - DNA, 21 bp, Artificial Sequence
  BRAF siRNA 253
cctatcgttagagtcttcctg